European Patent Application EP 4 566 673 A1, published June 11, 2025. Title: ANTIGEN-BINDING MOLECULE SPECIFICALLY BINDING TO GUCY2C AND CD3 AND PHARMACEUTICAL USE THEREOF. Applicant: JIANGSU HENGRUI PHARMACEUTICALS CO., LTD. Application IB PCT/CN2023/111149, filed August 4, 2023. The sequence listing filed with the application follows.

SEQUENCE LISTING (357 sequences)

SEQ ID NO: 1 - protein, 1073 aa, Homo sapiens
  CHAIN 1..1073: note = human GUCY2C
MKTLLLDLALWSLLFQPGWLSFSSQVSQNCHNGSYEISVLMMGNSAFAEPLKNLEDAVNEGLEIVRGRLQNAGLNVTVNATFMYSDGLIHNSGDCRSSTCEGLDLLRKISNAQRMGCVLIGPSCTYSTFQMYLDTELSYPMISAGSFGLSCDYKETLTRLMSPARKLMYFLVNFWKTNDLPFKTYSWSTSYVYKNGTETEDCFWYLNALEASVSYFSHELGFKVVLRQDKEFQDILMDHNRKSNVIIMCGGPEFLYKLKGDRAVAEDIVIILVDLFNDQYFEDNVTAPDYMKNVLVLTLSPGNSLLNSSFSRNLSPTKRDFALAYLNGILLFGHMLKIFLENGENITTPKFAHAFRNLTFEGYDGPVTLDDWGDVDSTMVLLYTSVDTKKYKVLLTYDTHVNKTYPVDMSPTFTWKNSKLPNDITGRGPQILMIAVFTLTGAVVLLLLVALLMLRKYRKDYELRQKKWSHIPPENIFPLETNETNHVSLKIDDDKRRDTIQRLRQCKYDKKRVILKDLKHNDGNFTEKQKIELNKLLQIDYYNLTKFYGTVKLDTMIFGVIEYCERGSLREVLNDTISYPDGTFMDWEFKISVLYDIAKGMSYLHSSKTEVHGRLKSTNCVVDSRMVVKITDFGCNSILPPKKDLWTAPEHLRQANISQKGDVYSYGIIAQEIILRKETFYTLSCRDRNEKIFRVENSNGMKPFRPDLFLETAEEKELEVYLLVKNCWEEDPEKRPDFKKIETTLAKIFGLFHDQKNESYMDTLIRRLQLYSRNLEHLVEERTQLYKAERDRADRLNFMLLPRLVVKSLKEKGFVEPELYEEVTIYFSDIVGFTTICKYSTPMEVVDMLNDIYKSFDHIVDHHDVYKVETIGDAYMVASGLPKRNGNRHAIDIAKMALEILSFMGTFELEHLPGLPIWIRIGVHSGPCAAGVVGIKMPRYCLFGDTVNTASRMESTGLPLRIHVSGSTIAILKRTECQFLYEVRGETYLKGRGNETTYWLTGMKDQKFNLPTPPTVENQQRLQAEFSDMIANSLQKRQAAGIRSQKPRRVASYKKGTLEYLQLNTTDKESTYF

SEQ ID NO: 2 - protein, 639 aa, synthetic construct
  CHAIN 1..639: note = hGUCY2C ECD-hFc
SQVSQNCHNGSYEISVLMMGNSAFAEPLKNLEDAVNEGLEIVRGRLQNAGLNVTVNATFMYSDGLIHNSGDCRSSTCEGLDLLRKISNAQRMGCVLIGPSCTYSTFQMYLDTELSYPMISAGSFGLSCDYKETLTRLMSPARKLMYFLVNFWKTNDLPFKTYSWSTSYVYKNGTETEDCFWYLNALEASVSYFSHELGFKVVLRQDKEFQDILMDHNRKSNVIIMCGGPEFLYKLKGDRAVAEDIVIILVDLFNDQYFEDNVTAPDYMKNVLVLTLSPGNSLLNSSFSRNLSPTKRDFALAYLNGILLFGHMLKIFLENGENITTPKFAHAFRNLTFEGYDGPVTLDDWGDVDSTMVLLYTSVDTKKYKVLLTYDTHVNKTYPVDMSPTFTWKNSKLPNDITGRGPQEPKSSDKTHTCPPCPAPELLGGPSVFLFPPKPKDTLMISRTPEVTCVVVDVSHEDPEVKFNWYVDGVEVHNAKTKPREEQYNSTYRVVSVLTVLHQDWLNGKEYKCKVSNKALPAPIEKTISKAKGQPREPQVYTLPPSRDELTKNQVSLTCLVKGFYPSDIAVEWESNGQPENNYKTTPPVLDSDGSFFLYSKLTVDKSRWQQGNVFSCSVMHEALHNHYTQKSLSLSPGK

SEQ ID NO: 3 - protein, 413 aa, synthetic construct
  CHAIN 1..413: note = hGUCY2C ECD-His
SQVSQNCHNGSYEISVLMMGNSAFAEPLKNLEDAVNEGLEIVRGRLQNAGLNVTVNATFMYSDGLIHNSGDCRSSTCEGLDLLRKISNAQRMGCVLIGPSCTYSTFQMYLDTELSYPMISAGSFGLSCDYKETLTRLMSPARKLMYFLVNFWKTNDLPFKTYSWSTSYVYKNGTETEDCFWYLNALEASVSYFSHELGFKVVLRQDKEFQDILMDHNRKSNVIIMCGGPEFLYKLKGDRAVAEDIVIILVDLFNDQYFEDNVTAPDYMKNVLVLTLSPGNSLLNSSFSRNLSPTKRDFALAYLNGILLFGHMLKIFLENGENITTPKFAHAFRNLTFEGYDGPVTLDDWGDVDSTMVLLYTSVDTKKYKVLLTYDTHVNKTYPVDMSPTFTWKNSKLPNDITGRGPQHHHHHH

SEQ ID NO: 4 - protein, 5 aa, synthetic construct
  DOMAIN 1..5: note = M81-HCDR1
DHNMN

SEQ ID NO: 5 - protein, 17 aa, synthetic construct
  DOMAIN 1..17: note = M81-HCDR2
VMNPKFGTINYNQKFKD

SEQ ID NO: 6 - protein, 9 aa, synthetic construct
  DOMAIN 1..9: note = M81-HCDR3
DDYPNYFDY

SEQ ID NO: 7 - protein, 10 aa, synthetic construct
  DOMAIN 1..10: note = M81-LCDR1
SASSSVNYMY

SEQ ID NO: 8 - protein, 7 aa, synthetic construct
  DOMAIN 1..7: note = M81-LCDR2
RTSNLAS

SEQ ID NO: 9 - protein, 9 aa, synthetic construct
  DOMAIN 1..9: note = M81-LCDR3
QQYHDYPPT

SEQ ID NO: 10 - protein, 5 aa, synthetic construct
  DOMAIN 1..5: note = M146-HCDR1
DYNMN

SEQ ID NO: 11 - protein, 17 aa, synthetic construct
  DOMAIN 1..17: note = M146-HCDR2
LINPKYGTTNYNQKFKG

SEQ ID NO: 12 - protein, 9 aa, synthetic construct
  DOMAIN 1..9: note = M146-HCDR3
DDYPAWFAY

SEQ ID NO: 13 - protein, 10 aa, synthetic construct
  DOMAIN 1..10: note = M146-LCDR1
SASSSLNYMY

SEQ ID NO: 14 - protein, 9 aa, synthetic construct
  DOMAIN 1..9: note = M146-LCDR3
QQYHSYPPT

SEQ ID NO: 15 - protein, 118 aa, synthetic construct
  DOMAIN 1..118: note = M81 VH
EFQLQQSGPELVKPGASVKISCKASGYSFTDHNMNWVKQSNGKSLEWIGVMNPKFGTINYNQKFKDKATLTVDQSSSTAYMQLNSLTSEDSAVYYCVRDDYPNYFDYWGQGTTLTVSS

SEQ ID NO: 16 - protein, 106 aa, synthetic construct
  DOMAIN 1..106: note = M81 VL
QIVLTQSPAIMSASPGEKVTISCSASSSVNYMYWYQQKPGSSPKSWIYRTSNLASGVSARFSGSGSGTSYSLTISSMEAEDAATYYCQQYHDYPPTFGGGTKLEIK

SEQ ID NO: 17 - protein, 118 aa, synthetic construct
  DOMAIN 1..118: note = M146 VH
EFQLQQSGPELVKPGASVKISCKASGYSFTDYNMNWVKQSNGKSLEWIGLINPKYGTTNYNQKFKGKATLTVDQSSSTAYMQLNSLTSEDSAVYYCAIDDYPAWFAYWGQGTLVTVSA

SEQ ID NO: 18 - protein, 106 aa, synthetic construct
  DOMAIN 1..106: note = M146 VL
QIVLTQSPAIMSASPGEKVTISCSASSSLNYMYWYQQKPGSSPKSWIYRTSNLASGVPARFSGSGSGTSYSLTISSMEAEDAATYYCQQYHSYPPTFGAGTKLELK

SEQ ID NO: 19 - protein, 5 aa, synthetic construct
  DOMAIN 1..5: note = P3-C7-HCDR1
DHYIH

SEQ ID NO: 20 - protein, 17 aa, synthetic construct
  DOMAIN 1..17: note = P3-C7-HCDR2
VINPYNDGATYNQKFKG

SEQ ID NO: 21 - protein, 11 aa, synthetic construct
  DOMAIN 1..11: note = P3-C7-HCDR3
PPRAYGNYAGY

SEQ ID NO: 22 - protein, 16 aa, synthetic construct
  DOMAIN 1..16: note = P3-C7-LCDR1
RSSQSLVHSNGNTYLH

SEQ ID NO: 23 - protein, 7 aa, synthetic construct
  DOMAIN 1..7: note = P3-C7-LCDR2
KVSNRFS

SEQ ID NO: 24 - protein, 9 aa, synthetic construct
  DOMAIN 1..9: note = P3-C7-LCDR3
SQSTHVPYT

SEQ ID NO: 25 - protein, 120 aa, synthetic construct
  DOMAIN 1..120: note = P3-C7 VH
EVQLQQSGPVLLKPGASVKMSCKASGYTFTDHYIHWVKLSHGKSLEWIGVINPYNDGATYNQKFKGKATLTVDKSSSTAYMELNSLTSEDSAVYYCARPPRAYGNYAGYWGQGTTLTVSS

SEQ ID NO: 26 - protein, 112 aa, synthetic construct
  DOMAIN 1..112: note = P3-C7 VL
DVVMTQTPLSLPVSLGDQASISCRSSQSLVHSNGNTYLHWYLQKPGQSPKLLIYKVSNRFSGVPDRFIGSGSRTDFTLKISRVEAEDLGVYFCSQSTHVPYTFGGGTRLEIK

SEQ ID NO: 27 - protein, 9 aa, synthetic construct
  DOMAIN 1..9: note = h81 H1-HCDR3
DNYPNYFDY

SEQ ID NO: 28 - protein, 7 aa, synthetic construct
  DOMAIN 1..7: note = h81 L4-LCDR2
RTSNDAS

SEQ ID NO: 29 - protein, 7 aa, synthetic construct
  DOMAIN 1..7: note = h81 L5-LCDR2
RTSNLAQ

SEQ ID NO: 30 - protein, 7 aa, synthetic construct
  DOMAIN 1..7: note = h81 L6-LCDR2
RTQNLAS

SEQ ID NO: 31 - protein, 106 aa, synthetic construct
  DOMAIN 1..106: note = h81 L1
EIVLTQSPATLSLSPGERATLSCSASSSVNYMYWYQQKPGQAPKSWIYRTSNLASGVPARFSGSGSGTDYTLTISSLEPEDFAVYYCQQYHDYPPTFGGGTKVEIK

SEQ ID NO: 32 - protein, 106 aa, synthetic construct
  DOMAIN 1..106: note = h81 L2
EIVLTQSPDFQSVTPGEKVTITCSASSSVNYMYWYQQKPDQSPKSWIYRTSNLASGVPSRFSGSGSGTDFTLTISSLEAEDAATYYCQQYHDYPPTFGGGTKVEIK

SEQ ID NO: 33 - protein, 106 aa, synthetic construct
  DOMAIN 1..106: note = h81 L3
DIQLTQSPSFLSASPGDRVTITCSASSSVNYMYWYQQKPGSSPKSWIYRTSNLASGVPSRFSGSGSGTEYTLTISSLQPEDFATYYCQQYHDYPPTFGGGTKVEIK

SEQ ID NO: 34 - protein, 106 aa, synthetic construct
  DOMAIN 1..106: note = h81 L4
DIQLTQSPSFLSASPGDRVTITCSASSSVNYMYWYQQKPGSSPKSWIYRTSNDASGVPSRFSGSGSGTEYTLTISSLQPEDFATYYCQQYHDYPPTFGGGTKVEIK

SEQ ID NO: 35 - protein, 106 aa, synthetic construct
  DOMAIN 1..106: note = h81 L5
DIQLTQSPSFLSASPGDRVTITCSASSSVNYMYWYQQKPGSSPKSWIYRTSNLAQGVPSRFSGSGSGTEYTLTISSLQPEDFATYYCQQYHDYPPTFGGGTKVEIK

SEQ ID NO: 36 - protein, 106 aa, synthetic construct
  DOMAIN 1..106: note = h81 L6
DIQLTQSPSFLSASPGDRVTITCSASSSVNYMYWYQQKPGSSPKSWIYRTQNLASGVPSRFSGSGSGTEYTLTISSLQPEDFATYYCQQYHDYPPTFGGGTKVEIK

SEQ ID NO: 37 - protein, 118 aa, synthetic construct
  DOMAIN 1..118: note = h81 H1
EVQLVQSGAEVKKPGASVKVSCKASGYTFTDHNMNWVKQAPGQRLEWMGVMNPKFGTINYNQKFKDKATITRDTSASTAYMELSSLRSEDTAVYYCARDNYPNYFDYWGQGTTVTVSS

SEQ ID NO: 38 - protein, 118 aa, synthetic construct
  DOMAIN 1..118: note = h81 H2
EVQLVQSGAEVKKPGASVKVSCKASGYTFTDHNMNWVKQAPGQRLEWMGVMNPKFGTINYNQKFKDKATITRDTSASTAYMELSSLRSEDTAVYYCARDDYPNYFDYWGQGTTVTVSS

SEQ ID NO: 39 - protein, 7 aa, synthetic construct
  DOMAIN 1..7: note = h146 L1-LCDR2
RTSQLAS

SEQ ID NO: 40 - protein, 9 aa, synthetic construct
  DOMAIN 1..9: note = h146 H1-HCDR3
DNYPAWFAY

SEQ ID NO: 41 - protein, 106 aa, synthetic construct
  DOMAIN 1..106: note = h146 L1
EIVLTQSPATLSLSPGERATLSCSASSSLNYMYWYQQKPGSSPRPWIYRTSQLASGVPARFSGSGSGTDYTLTISSLEPEDFAVYYCQQYHSYPPTFGGGTKVEIK

SEQ ID NO: 42 - protein, 118 aa, synthetic construct
  DOMAIN 1..118: note = h146 H1
EFQLVQSGAEVKKPGASVKVSCKASGYSFTDYNMNWVRQAPGQRLEWMGLINPKYGTTNYNQKFKGRVTLTVDQSSSTAYMELSSLRSEDTAVYYCARDNYPAWFAYWGQGTTVTVSS

SEQ ID NO: 43 - protein, 16 aa, synthetic construct
  DOMAIN 1..16: note = hP3-C7 L3-LCDR1
RSSQSLVHSQGNTYLH

SEQ ID NO: 44 - protein, 16 aa, synthetic construct
  DOMAIN 1..16: note = hP3-C7 L4-LCDR1
RSSQSLVHSSGNTYLH

SEQ ID NO: 45 - protein, 16 aa, synthetic construct
  DOMAIN 1..16: note = hP3-C7 L5-LCDR1
RSSQSLVHSTGNTYLH

SEQ ID NO: 46 - protein, 16 aa, synthetic construct
  DOMAIN 1..16: note = hP3-C7 L6-LCDR1
RSSQSLVHSNVNTYLH

SEQ ID NO: 47 - protein, 16 aa, synthetic construct
  DOMAIN 1..16: note = hP3-C7 L7/hP3-C7 L8-LCDR1
RSSQSLVHSNQNTYLH

SEQ ID NO: 48 - protein, 112 aa, synthetic construct
  DOMAIN 1..112: note = hP3-C7 L1
DIVMTQTPLSLPVTPGEPASISCRSSQSLVHSNGNTYLHWYLQKPGQSPQLLIYKVSNRFSGVPDRFSGSGSGTDFTLKISRVEAEDVGVYYCSQSTHVPYTFGGGTKVEIK

SEQ ID NO: 49 - protein, 112 aa, synthetic construct
  DOMAIN 1..112: note = hP3-C7 L2
DVVMTQTPLSLPVTPGEPASISCRSSQSLVHSNGNTYLHWYLQKPGQSPQLLIYKVSNRFSGVPDRFSGSGSRTDFTLKISRVEAEDVGVYYCSQSTHVPYTFGGGTKVEIK

SEQ ID NO: 50 - protein, 112 aa, synthetic construct
  DOMAIN 1..112: note = hP3-C7 L3
DVVMTQTPLSLPVTPGEPASISCRSSQSLVHSQGNTYLHWYLQKPGQSPQLLIYKVSNRFSGVPDRFSGSGSRTDFTLKISRVEAEDVGVYYCSQSTHVPYTFGGGTKVEIK

SEQ ID NO: 51 - protein, 112 aa, synthetic construct
  DOMAIN 1..112: note = hP3-C7 L4
DVVMTQTPLSLPVTPGEPASISCRSSQSLVHSSGNTYLHWYLQKPGQSPQLLIYKVSNRFSGVPDRFSGSGSRTDFTLKISRVEAEDVGVYYCSQSTHVPYTFGGGTKVEIK

SEQ ID NO: 52 - protein, 112 aa, synthetic construct
  DOMAIN 1..112: note = hP3-C7 L5
DVVMTQTPLSLPVTPGEPASISCRSSQSLVHSTGNTYLHWYLQKPGQSPQLLIYKVSNRFSGVPDRFSGSGSRTDFTLKISRVEAEDVGVYYCSQSTHVPYTFGGGTKVEIK

SEQ ID NO: 53 - protein, 112 aa, synthetic construct
  DOMAIN 1..112: note = hP3-C7 L5
DVVMTQTPLSLPVTPGEPASISCRSSQSLVHSNVNTYLHWYLQKPGQSPQLLIYKVSNRFSGVPDRFSGSGSRTDFTLKISRVEAEDVGVYYCSQSTHVPYTFGGGTKVEIK

SEQ ID NO: 54 - protein, 112 aa, synthetic construct
  DOMAIN 1..112: note = hP3-C7 L7
DVVMTQTPLSLPVTPGEPASISCRSSQSLVHSNQNTYLHWYLQKPGQSPQLLIYKVSNRFSGVPDRFSGSGSRTDFTLKISRVEAEDVGVYYCSQSTHVPYTFGGGTKVEIK

SEQ ID NO: 55 - protein, 112 aa, synthetic construct
  DOMAIN 1..112: note = hP3-C7 L8
DVVMTQSPSSLSASVGDRVTITCRSSQSLVHSNQNTYLHWYQQKPGKAPKLLIYKVSNRFSGVPSRFSGSGSRTDFTLKISSLQPEDFATYYCSQSTHVPYTFGGGTKVEIK

SEQ ID NO: 56 - protein, 120 aa, synthetic construct
  DOMAIN 1..120: note = hP3-C7 H1
EVQLVQSGAEVKKPGASVKVSCKASGYTFTDHYIHWVRQAPGQGLEWMGVINPYNDGATYNQKFKGRVTMTVDKSTSTVYMELSSLRSEDTAVYYCARPPRAYGNYAGYWGQGTTVTVSS

SEQ ID NO: 57 - protein, 120 aa, synthetic construct
  DOMAIN 1..120: note = hP3-C7 H2
EVQLVQSGAEVKKPGASVKVSCKASGYTFTDHYIHWVRLAPGKGLEWMGVINPYNDGATYNQKFKGRVTLTVDKSTSTVYMELSSLRSEDTAVYYCARPPRAYGNYAGYWGQGTTVTVSS

SEQ ID NO: 58 - protein, 330 aa, synthetic construct [sequence omitted]

SEQ ID NO: 59 - protein, 107 aa, synthetic construct [sequence omitted]

SEQ ID NO: 60 - protein, 448 aa, synthetic construct
  CHAIN 1..448: note = 81 L3H1 heavy chain
EVQLVQSGAEVKKPGASVKVSCKASGYTFTDHNMNWVKQAPGQRLEWMGVMNPKFGTINYNQKFKDKATITRDTSASTAYMELSSLRSEDTAVYYCARDNYPNYFDYWGQGTTVTVSSASTKGPSVFPLAPSSKSTSGGTAALGCLVKDYFPEPVTVSWNSGALTSGVHTFPAVLQSSGLYSLSSVVTVPSSSLGTQTYICNVNHKPSNTKVDKKVEPKSCDKTHTCPPCPAPELLGGPSVFLFPPKPKDTLMISRTPEVTCVVVDVSHEDPEVKFNWYVDGVEVHNAKTKPREEQYNSTYRVVSVLTVLHQDWLNGKEYKCKVSNKALPAPIEKTISKAKGQPREPQVYTLPPSRDELTKNQVSLTCLVKGFYPSDIAVEWESNGQPENNYKTTPPVLDSDGSFFLYSKLTVDKSRWQQGNVFSCSVMHEALHNHYTQKSLSLSPGK

SEQ ID NO: 61 - protein, 213 aa, synthetic construct
  CHAIN 1..213: note = 81 L3H1 light chain
DIQLTQSPSFLSASPGDRVTITCSASSSVNYMYWYQQKPGSSPKSWIYRTSNLASGVPSRFSGSGSGTEYTLTISSLQPEDFATYYCQQYHDYPPTFGGGTKVEIKRTVAAPSVFIFPPSDEQLKSGTASVVCLLNNFYPREAKVQWKVDNALQSGNSQESVTEQDSKDSTYSLSSTLTLSKADYEKHKVYACEVTHQGLSSPVTKSFNRGEC

SEQ ID NO: 62 - protein, 448 aa, synthetic construct
  CHAIN 1..448: note = 146 L1H1 heavy chain
EFQLVQSGAEVKKPGASVKVSCKASGYSFTDYNMNWVRQAPGQRLEWMGLINPKYGTTNYNQKFKGRVTLTVDQSSSTAYMELSSLRSEDTAVYYCARDNYPAWFAYWGQGTTVTVSSASTKGPSVFPLAPSSKSTSGGTAALGCLVKDYFPEPVTVSWNSGALTSGVHTFPAVLQSSGLYSLSSVVTVPSSSLGTQTYICNVNHKPSNTKVDKKVEPKSCDKTHTCPPCPAPELLGGPSVFLFPPKPKDTLMISRTPEVTCVVVDVSHEDPEVKFNWYVDGVEVHNAKTKPREEQYNSTYRVVSVLTVLHQDWLNGKEYKCKVSNKALPAPIEKTISKAKGQPREPQVYTLPPSRDELTKNQVSLTCLVKGFYPSDIAVEWESNGQPENNYKTTPPVLDSDGSFFLYSKLTVDKSRWQQGNVFSCSVMHEALHNHYTQKSLSLSPGK

SEQ ID NO: 63 - protein, 213 aa, synthetic construct
  CHAIN 1..213: note = 146 L1H1 light chain
EIVLTQSPATLSLSPGERATLSCSASSSLNYMYWYQQKPGSSPRPWIYRTSQLASGVPARFSGSGSGTDYTLTISSLEPEDFAVYYCQQYHSYPPTFGGGTKVEIKRTVAAPSVFIFPPSDEQLKSGTASVVCLLNNFYPREAKVQWKVDNALQSGNSQESVTEQDSKDSTYSLSSTLTLSKADYEKHKVYACEVTHQGLSSPVTKSFNRGEC

SEQ ID NO: 64 - protein, 450 aa, synthetic construct
  CHAIN 1..450: note = P3-C7 L7H1 heavy chain
EVQLVQSGAEVKKPGASVKVSCKASGYTFTDHYIHWVRQAPGQGLEWMGVINPYNDGATYNQKFKGRVTMTVDKSTSTVYMELSSLRSEDTAVYYCARPPRAYGNYAGYWGQGTTVTVSSASTKGPSVFPLAPSSKSTSGGTAALGCLVKDYFPEPVTVSWNSGALTSGVHTFPAVLQSSGLYSLSSVVTVPSSSLGTQTYICNVNHKPSNTKVDKKVEPKSCDKTHTCPPCPAPELLGGPSVFLFPPKPKDTLMISRTPEVTCVVVDVSHEDPEVKFNWYVDGVEVHNAKTKPREEQYNSTYRVVSVLTVLHQDWLNGKEYKCKVSNKALPAPIEKTISKAKGQPREPQVYTLPPSRDELTKNQVSLTCLVKGFYPSDIAVEWESNGQPENNYKTTPPVLDSDGSFFLYSKLTVDKSRWQQGNVFSCSVMHEALHNHYTQKSLSLSPGK

SEQ ID NO: 65 - protein, 219 aa, synthetic construct
  CHAIN 1..219: note = P3-C7 L7H1 light chain
DVVMTQTPLSLPVTPGEPASISCRSSQSLVHSNQNTYLHWYLQKPGQSPQLLIYKVSNRFSGVPDRFSGSGSRTDFTLKISRVEAEDVGVYYCSQSTHVPYTFGGGTKVEIKRTVAAPSVFIFPPSDEQLKSGTASVVCLLNNFYPREAKVQWKVDNALQSGNSQESVTEQDSKDSTYSLSSTLTLSKADYEKHKVYACEVTHQGLSSPVTKSFNRGEC

SEQ ID NO: 66 - protein, 219 aa, synthetic construct
  CHAIN 1..219: note = P3-C7 L8H1 light chain
DVVMTQSPSSLSASVGDRVTITCRSSQSLVHSNQNTYLHWYQQKPGKAPKLLIYKVSNRFSGVPSRFSGSGSRTDFTLKISSLQPEDFATYYCSQSTHVPYTFGGGTKVEIKRTVAAPSVFIFPPSDEQLKSGTASVVCLLNNFYPREAKVQWKVDNALQSGNSQESVTEQDSKDSTYSLSSTLTLSKADYEKHKVYACEVTHQGLSSPVTKSFNRGEC

SEQ ID NO: 67 - protein, 452 aa, synthetic construct
  CHAIN 1..452: note = 1608 heavy chain
EVQLVESGGGLVQPGGSLRLSCAASGFTFSSYWMHWVRQAPGKGLEWIGEIKPSNELTNVHEKFKDRFTISVDKAKNSAYLQMNSLRAEDTAVYYCTRTITTTEGYWFFDVWGQGTLVTVSSASTKGPSVFPLAPSSKSTSGGTAALGCLVKDYFPEPVTVSWNSGALTSGVHTFPAVLQSSGLYSLSSVVTVPSSSLGTQTYICNVNHKPSNTKVDKKVEPKSCDKTHTCPPCPAPELLGGPSVFLFPPKPKDTLMISRTPEVTCVVVDVSHEDPEVKFNWYVDGVEVHNAKTKPREEQYNSTYRVVSVLTVLHQDWLNGKEYKCKVSNKALPAPIEKTISKAKGQPREPQVYTLPPSRDELTKNQVSLTCLVKGFYPSDIAVEWESNGQPENNYKTTPPVLDSDGSFFLYSKLTVDKSRWQQGNVFSCSVMHEALHNHYTQKSLSLSPGK

SEQ ID NO: 68 - protein, 217 aa, synthetic construct
  CHAIN 1..217: note = 1608 light chain
DIQLTQSPSSLSASVGDRVTITCRASESVDYYGSSLLQWYQQKPGKAPKLLIYAASKLASGVPSRFSGSGSGTDFTLTISSLQPEDFATYYCQQTRKAYTFGQGTKLEIKRTVAAPSVFIFPPSDEQLKSGTASVVCLLNNFYPREAKVQWKVDNALQSGNSQESVTEQDSKDSTYSLSSTLTLSKADYEKHKVYACEVTHQGLSSPVTKSFNRGEC

SEQ ID NO: 69 - protein, 449 aa, synthetic construct
  CHAIN 1..449: note = 5F9-HC
QVQLQQWGAGLLKPSETLSLTCAVFGGSFSGYYWSWIRQPPGKGLEWIGEINHRGNTNDNPSLKSRVTISVDTSKNQFALKLSSVTAADTAVYYCARERGYTYGNFDHWGQGTLVTVSSASTKGPSVFPLAPSSKSTSGGTAALGCLVKDYFPEPVTVSWNSGALTSGVHTFPAVLQSSGLYSLSSVVTVPSSSLGTQTYICNVNHKPSNTKVDKKVEPKSCDKTHTCPPCPAPELLGGPSVFLFPPKPKDTLMISRTPEVTCVVVDVSHEDPEVKFNWYVDGVEVHNAKTKPREEQYNSTYRVVSVLTVLHQDWLNGKEYKCKVSNKALPAPIEKTISKAKGQPREPQVYTLPPSRDELTKNQVSLTCLVKGFYPSDIAVEWESNGQPENNYKTTPPVLDSDGSFFLYSKLTVDKSRWQQGNVFSCSVMHEALHNHYTQKSLSLSPGK

SEQ ID NO: 70 - protein, 214 aa, synthetic construct
  CHAIN 1..214: note = 5F9-LC
EIVMTQSPATLSVSPGERATLSCRASQSVSRNLAWYQQKPGQAPRLLIYGASTRATGIPARFSGSGSGTEFTLTIGSLQSEDFAVYYCQQYKTWPRTFGQGTNVEIKRTVAAPSVFIFPPSDEQLKSGTASVVCLLNNFYPREAKVQWKVDNALQSGNSQESVTEQDSKDSTYSLSSTLTLSKADYEKHKVYACEVTHQGLSSPVTKSFNRGEC

SEQ ID NO: 71 - protein, 5 aa, synthetic construct
  DOMAIN 1..5: note = S107E-HCDR1
KYAMN

SEQ ID NO: 72 - protein, 19 aa, synthetic construct
  DOMAIN 1..19: note = S107E-HCDR2
RIRSKYNNYATYYADSVKD

SEQ ID NO: 73 - protein, 14 aa, synthetic construct
  DOMAIN 1..14: note = S107E-HCDR3
HGNFGNEYISYWAY

SEQ ID NO: 74 - protein, 14 aa, synthetic construct
  DOMAIN 1..14: note = S107E-LCDR1
GSSTGAVTSGNYPN

SEQ ID NO: 75 - protein, 7 aa, synthetic construct
  DOMAIN 1..7: note = S107E-LCDR2
GTKFLAP

SEQ ID NO: 76 - protein, 9 aa, synthetic construct
  DOMAIN 1..9: note = S107E-LCDR3
VLWYSNRWV

SEQ ID NO: 77 - protein, 125 aa, synthetic construct
  DOMAIN 1..125: note = S107E-VH
EVQLVESGGGLVQPGGSLKLSCAASGFTFNKYAMNWVRQAPGKGLEWVARIRSKYNNYATYYADSVKDRFTISRDDSKNTAYLQMNNLKTEDTAVYYCVRHGNFGNEYISYWAYWGQGTLVTVSS

SEQ ID NO: 78 - protein, 109 aa, synthetic construct
  DOMAIN 1..109: note = S107E-VL
QTVVTQEPSLTVSPGGTVTLTCGSSTGAVTSGNYPNWVQQKPGQAPRGLIGGTKFLAPGTPARFSGSLLGGKAALTLSGVQPEDEAEYYCVLWYSNRWVFGGGTKLTVL

SEQ ID NO: 79 - protein, 221 aa, synthetic construct
  DOMAIN 1..221: note = IgG1Fc(Knob-DI L234A/L235A/G237A/Y349C/T366W)
CPPCPAPEAAGAPSVFLFPPKPKDTLMISRTPEVTCVVVDVSHEDPEVKFNWYVDGVEVHNAKTKPREEQYNSTYRVVSVLTVLHQDWLNGKEYKCKVSNKALPAPIEKTISKAKGQPREPQVCTLPPSREEMTKNQVSLWCLVKGFYPSDIAVEWESNGQPENNYKTTPPVLDSDGSFFLYSKLTVDKSRWQQGNVFSCSVMHEALHNHYTQKSLSLSPG

SEQ ID NO: 80 - protein, 221 aa, synthetic construct
  DOMAIN 1..221: note = IgG1Fc(Hole-DI L234A/L235A/G237A/S354C/T366S/L368A/Y407V)
CPPCPAPEAAGAPSVFLFPPKPKDTLMISRTPEVTCVVVDVSHEDPEVKFNWYVDGVEVHNAKTKPREEQYNSTYRVVSVLTVLHQDWLNGKEYKCKVSNKALPAPIEKTISKAKGQPREPQVYTLPPCREEMTKNQVSLSCAVKGFYPSDIAVEWESNGQPENNYKTTPPVLDSDGSFFLVSKLTVDKSRWQQGNVFSCSVMHEALHNHYTQKSLSLSPG

SEQ ID NO: 81 - protein, 8 aa, synthetic construct
  DOMAIN 1..8: note = linker1
GGGSGGGG

SEQ ID NO: 82 - skipped

SEQ ID NO: 83 - protein, 9 aa, synthetic construct
  DOMAIN 1..9: note = linker3
GGGGSGGGG

SEQ ID NO: 84 - protein, 103 aa, synthetic construct
  DOMAIN 1..103: note = IgG1(CH1)
ASTKGPSVFPLAPSSKSTSGGTAALGCLVKDYFPEPVTVSWNSGALTSGVHTFPAVLQSSGLYSLSSVVTVPSSSLGTQTYICNVNHKPSNTKVDKKVEPKSC

SEQ ID NO: 85 - protein, 227 aa, synthetic construct
  DOMAIN 1..227: note = IgG1Fc(Knob L234A/L235A/S354C/T366W)
DKTHTCPPCPAPEAAGGPSVFLFPPKPKDTLMISRTPEVTCVVVDVSHEDPEVKFNWYVDGVEVHNAKTKPREEQYNSTYRVVSVLTVLHQDWLNGKEYKCKVSNKALPAPIEKTISKAKGQPREPQVYTLPPCREEMTKNQVSLWCLVKGFYPSDIAVEWESNGQPENNYKTTPPVLDSDGSFFLYSKLTVDKSRWQQGNVFSCSVMHEALHNHYTQKSLSLSPGK

SEQ ID NO: 86 - protein, 227 aa, synthetic construct
  DOMAIN 1..227: note = IgG1Fc(Hole L234A/L235A/Y349C/T366S/L368A/Y407V)
DKTHTCPPCPAPEAAGGPSVFLFPPKPKDTLMISRTPEVTCVVVDVSHEDPEVKFNWYVDGVEVHNAKTKPREEQYNSTYRVVSVLTVLHQDWLNGKEYKCKVSNKALPAPIEKTISKAKGQPREPQVCTLPPSREEMTKNQVSLSCAVKGFYPSDIAVEWESNGQPENNYKTTPPVLDSDGSFFLVSKLTVDKSRWQQGNVFSCSVMHEALHNHYTQKSLSLSPGK

SEQ ID NO: 87 - protein, 105 aa, synthetic construct
  DOMAIN 1..105: note = CL(Lambda)
GQPKANPTVTLFPPSSEELQANKATLVCLISDFYPGAVTVAWKADGSPVKAGVETTKPSKQSNNKYAASSYLSLTPEQWKSHRSYSCQVTHEGSTVEKTVAPTEC

SEQ ID NO: 88 - protein, 14 aa, synthetic construct
  DOMAIN 1..14: note = N103Q N106Q-HCDR3
HGQFGQSYISYWAY

SEQ ID NO: 89 - protein, 125 aa, synthetic construct
  DOMAIN 1..125: note = N103QN106Q-VH
EVQLVESGGGLVQPGGSLKLSCAASGFTFNKYAMNWVRQAPGKGLEWVARIRSKYNNYATYYADSVKDRFTISRDDSKNTAYLQMNNLKTEDTAVYYCVRHGQFGQSYISYWAYWGQGTLVTVSS

SEQ ID NO: 90 - protein, 5 aa, synthetic construct
  DOMAIN 1..5: note = linker4
GGGGS

SEQ ID NO: 91 - protein, 455 aa, synthetic construct
  CHAIN 1..455: note = Format 2-1
EVQLVESGGGLVQPGGSLKLSCAASGFTFNKYAMNWVRQAPGKGLEWVARIRSKYNNYATYYADSVKDRFTISRDDSKNTAYLQMNNLKTEDTAVYYCVRHGNFGNEYISYWAYWGQGTLVTVSSASTKGPSVFPLAPSSKSTSGGTAALGCLVKDYFPEPVTVSWNSGALTSGVHTFPAVLQSSGLYSLSSVVTVPSSSLGTQTYICNVNHKPSNTKVDKKVEPKSCDKTHTCPPCPAPEAAGGPSVFLFPPKPKDTLMISRTPEVTCVVVDVSHEDPEVKFNWYVDGVEVHNAKTKPREEQYNSTYRVVSVLTVLHQDWLNGKEYKCKVSNKALPAPIEKTISKAKGQPREPQVYTLPPCREEMTKNQVSLWCLVKGFYPSDIAVEWESNGQPENNYKTTPPVLDSDGSFFLYSKLTVDKSRWQQGNVFSCSVMHEALHNHYTQKSLSLSPGK

SEQ ID NO: 92 - protein, 214 aa, synthetic construct
  CHAIN 1..214: note = Format 2-2
QTVVTQEPSLTVSPGGTVTLTCGSSTGAVTSGNYPNWVQQKPGQAPRGLIGGTKFLAPGTPARFSGSLLGGKAALTLSGVQPEDEAEYYCVLWYSNRWVFGGGTKLTVLGQPKANPTVTLFPPSSEELQANKATLVCLISDFYPGAVTVAWKADGSPVKAGVETTKPSKQSNNKYAASSYLSLTPEQWKSHRSYSCQVTHEGSTVEKTVAPTEC

SEQ ID NO: 93 - protein, 455 aa, synthetic construct
  CHAIN 1..455: note = Format 3-3
EVQLVESGGGLVQPGGSLKLSCAASGFTFNKYAMNWVRQAPGKGLEWVARIRSKYNNYATYYADSVKDRFTISRDDSKNTAYLQMNNLKTEDTAVYYCVRHGNFGNEYISYWAYWGQGTLVTVSSASTKGPSVFPLAPSSKSTSGGTAALGCLVKDYFPEPVTVSWNSGALTSGVHTFPAVLQSSGLYSLSSVVTVPSSSLGTQTYICNVNHKPSNTKVDKKVEPKSCDKTHTCPPCPAPEAAGGPSVFLFPPKPKDTLMISRTPEVTCVVVDVSHEDPEVKFNWYVDGVEVHNAKTKPREEQYNSTYRVVSVLTVLHQDWLNGKEYKCKVSNKALPAPIEKTISKAKGQPREPQVCTLPPSREEMTKNQVSLSCAVKGFYPSDIAVEWESNGQPENNYKTTPPVLDSDGSFFLVSKLTVDKSRWQQGNVFSCSVMHEALHNHYTQKSLSLSPGK

SEQ ID NO: 94 - protein, 227 aa, synthetic construct
  DOMAIN 1..227: note = IgG1Fc (L234A/L235A)
DKTHTCPPCPAPEAAGGPSVFLFPPKPKDTLMISRTPEVTCVVVDVSHEDPEVKFNWYVDGVEVHNAKTKPREEQYNSTYRVVSVLTVLHQDWLNGKEYKCKVSNKALPAPIEKTISKAKGQPREPQVYTLPPSREEMTKNQVSLTCLVKGFYPSDIAVEWESNGQPENNYKTTPPVLDSDGSFFLYSKLTVDKSRWQQGNVFSCSVMHEALHNHYTQKSLSLSPGK

SEQ ID NO: 95 - protein, 15 aa, synthetic construct
  DOMAIN 1..15: note = linker5
GGGGSGGGGSGGGGS

SEQ ID NO: 96 - skipped

SEQ ID NO: 97 - protein, 10 aa, synthetic construct
  DOMAIN 1..10: note = linker7
GGGGSGGGGS

SEQ ID NO: 98 - protein, 212 aa, synthetic construct
  CHAIN 1..212: note = Format 5-3
QTVVTQEPSLTVSPGGTVTLTCGSSTGAVTSGNYPNWVQQKPGQAPRGLIGGTKFLAPGTPARFSGSLLGGKAALTLSGVQPEDEAEYYCVLWYSNRWVFGGGTKLTVLGGGGSGIPPKIECLPIDISIDEGKVLTVASAFTGEPTPEVTWSTGGRKIHSQEQGRFHIENTDDSTTLTIKDVQKQDGGLYTLTLRNEFGSDSATVNIHIRSI

SEQ ID NO: 99 - protein, 467 aa, synthetic construct
  CHAIN 1..467: note = P3-C7 L7H1-1-1
DVVMTQTPLSLPVTPGEPASISCRSSQSLVHSNQNTYLHWYLQKPGQSPQLLIYKVSNRFSGVPDRFSGSGSRTDFTLKISRVEAEDVGVYYCSQSTHVPYTFGGGTKVEIKGGGSGGGGEVQLVESGGGLVQPGGSLKLSCAASGFTFNKYAMNWVRQAPGKGLEWVARIRSKYNNYATYYADSVKDRFTISRDDSKNTAYLQMNNLKTEDTAVYYCVRHGNFGNEYISYWAYWGQGTLVTVSSGCPPCPAPEAAGAPSVFLFPPKPKDTLMISRTPEVTCVVVDVSHEDPEVKFNWYVDGVEVHNAKTKPREEQYNSTYRVVSVLTVLHQDWLNGKEYKCKVSNKALPAPIEKTISKAKGQPREPQVCTLPPSREEMTKNQVSLWCLVKGFYPSDIAVEWESNGQPENNYKTTPPVLDSDGSFFLYSKLTVDKSRWQQGNVFSCSVMHEALHNHYTQKSLSLSPG

SEQ ID NO: 100 - protein, 460 aa, synthetic construct
  CHAIN 1..460: note = P3-C7 L7H1-1-2
QTVVTQEPSLTVSPGGTVTLTCGSSTGAVTSGNYPNWVQQKPGQAPRGLIGGTKFLAPGTPARFSGSLLGGKAALTLSGVQPEDEAEYYCVLWYSNRWVFGGGTKLTVLGGGGSGGGGEVQLVQSGAEVKKPGASVKVSCKASGYTFTDHYIHWVRQAPGQGLEWMGVINPYNDGATYNQKFKGRVTMTVDKSTSTVYMELSSLRSEDTAVYYCARPPRAYGNYAGYWGQGTTVTVSSGCPPCPAPEAAGAPSVFLFPPKPKDTLMISRTPEVTCVVVDVSHEDPEVKFNWYVDGVEVHNAKTKPREEQYNSTYRVVSVLTVLHQDWLNGKEYKCKVSNKALPAPIEKTISKAKGQPREPQVYTLPPCREEMTKNQVSLSCAVKGFYPSDIAVEWESNGQPENNYKTTPPVLDSDGSFFLVSKLTVDKSRWQQGNVFSCSVMHEALHNHYTQKSLSLSPG

SEQ ID NO: 101 - protein, 467 aa, synthetic construct
  CHAIN 1..467: note = P3-C7 L8H1-1-1
DVVMTQSPSSLSASVGDRVTITCRSSQSLVHSNQNTYLHWYQQKPGKAPKLLIYKVSNRFSGVPSRFSGSGSRTDFTLKISSLQPEDFATYYCSQSTHVPYTFGGGTKVEIKGGGSGGGGEVQLVESGGGLVQPGGSLKLSCAASGFTFNKYAMNWVRQAPGKGLEWVARIRSKYNNYATYYADSVKDRFTISRDDSKNTAYLQMNNLKTEDTAVYYCVRHGNFGNEYISYWAYWGQGTLVTVSSGCPPCPAPEAAGAPSVFLFPPKPKDTLMISRTPEVTCVVVDVSHEDPEVKFNWYVDGVEVHNAKTKPREEQYNSTYRVVSVLTVLHQDWLNGKEYKCKVSNKALPAPIEKTISKAKGQPREPQVCTLPPSREEMTKNQVSLWCLVKGFYPSDIAVEWESNGQPENNYKTTPPVLDSDGSFFLYSKLTVDKSRWQQGNVFSCSVMHEALHNHYTQKSLSLSPG

SEQ ID NO: 102 - protein, 461 aa, synthetic construct
  CHAIN 1..461: note = M81-1-1
QIVLTQSPAIMSASPGEKVTISCSASSSVNYMYWYQQKPGSSPKSWIYRTSNLASGVSARFSGSGSGTSYSLTISSMEAEDAATYYCQQYHDYPPTFGGGTKLEIKGGGSGGGGEVQLVESGGGLVQPGGSLKLSCAASGFTFNKYAMNWVRQAPGKGLEWVARIRSKYNNYATYYADSVKDRFTISRDDSKNTAYLQMNNLKTEDTAVYYCVRHGNFGNEYISYWAYWGQGTLVTVSSGCPPCPAPEAAGAPSVFLFPPKPKDTLMISRTPEVTCVVVDVSHEDPEVKFNWYVDGVEVHNAKTKPREEQYNSTYRVVSVLTVLHQDWLNGKEYKCKVSNKALPAPIEKTISKAKGQPREPQVCTLPPSREEMTKNQVSLWCLVKGFYPSDIAVEWESNGQPENNYKTTPPVLDSDGSFFLYSKLTVDKSRWQQGNVFSCSVMHEALHNHYTQKSLSLSPG

SEQ ID NO: 103 - protein, 458 aa, synthetic construct
  CHAIN 1..458: note = M81-1-2
QTVVTQEPSLTVSPGGTVTLTCGSSTGAVTSGNYPNWVQQKPGQAPRGLIGGTKFLAPGTPARFSGSLLGGKAALTLSGVQPEDEAEYYCVLWYSNRWVFGGGTKLTVLGGGGSGGGGEFQLQQSGPELVKPGASVKISCKASGYSFTDHNMNWVKQSNGKSLEWIGVMNPKFGTINYNQKFKDKATLTVDQSSSTAYMQLNSLTSEDSAVYYCVRDDYPNYFDYWGQGTTLTVSSGCPPCPAPEAAGAPSVFLFPPKPKDTLMISRTPEVTCVVVDVSHEDPEVKFNWYVDGVEVHNAKTKPREEQYNSTYRVVSVLTVLHQDWLNGKEYKCKVSNKALPAPIEKTISKAKGQPREPQVYTLPPCREEMTKNQVSLSCAVKGFYPSDIAVEWESNGQPENNYKTTPPVLDSDGSFFLVSKLTVDKSRWQQGNVFSCSVMHEALHNHYTQKSLSLSPG

SEQ ID NO: 104 - protein, 461 aa, synthetic construct
  CHAIN 1..461: note = M146-1-1
QIVLTQSPAIMSASPGEKVTISCSASSSLNYMYWYQQKPGSSPKSWIYRTSNLASGVPARFSGSGSGTSYSLTISSMEAEDAATYYCQQYHSYPPTFGAGTKLELKGGGSGGGGEVQLVESGGGLVQPGGSLKLSCAASGFTFNKYAMNWVRQAPGKGLEWVARIRSKYNNYATYYADSVKDRFTISRDDSKNTAYLQMNNLKTEDTAVYYCVRHGNFGNEYISYWAYWGQGTLVTVSSGCPPCPAPEAAGAPSVFLFPPKPKDTLMISRTPEVTCVVVDVSHEDPEVKFNWYVDGVEVHNAKTKPREEQYNSTYRVVSVLTVLHQDWLNGKEYKCKVSNKALPAPIEKTISKAKGQPREPQVCTLPPSREEMTKNQVSLWCLVKGFYPSDIAVEWESNGQPENNYKTTPPVLDSDGSFFLYSKLTVDKSRWQQGNVFSCSVMHEALHNHYTQKSLSLSPG

SEQ ID NO: 105 - protein, 458 aa, synthetic construct
  CHAIN 1..458: note = M146-1-2
QTVVTQEPSLTVSPGGTVTLTCGSSTGAVTSGNYPNWVQQKPGQAPRGLIGGTKFLAPGTPARFSGSLLGGKAALTLSGVQPEDEAEYYCVLWYSNRWVFGGGTKLTVLGGGGSGGGGEFQLQQSGPELVKPGASVKISCKASGYSFTDYNMNWVKQSNGKSLEWIGLINPKYGTTNYNQKFKGKATLTVDQSSSTAYMQLNSLTSEDSAVYYCAIDDYPAWFAYWGQGTLVTVSAGCPPCPAPEAAGAPSVFLFPPKPKDTLMISRTPEVTCVVVDVSHEDPEVKFNWYVDGVEVHNAKTKPREEQYNSTYRVVSVLTVLHQDWLNGKEYKCKVSNKALPAPIEKTISKAKGQPREPQVYTLPPCREEMTKNQVSLSCAVKGFYPSDIAVEWESNGQPENNYKTTPPVLDSDGSFFLVSKLTVDKSRWQQGNVFSCSVMHEALHNHYTQKSLSLSPG

SEQ ID NO: 106 - protein, 449 aa, synthetic construct
  CHAIN 1..449: note = P3-C7 L7H1-2-3
EVQLVQSGAEVKKPGASVKVSCKASGYTFTDHYIHWVRQAPGQGLEWMGVINPYNDGATYNQKFKGRVTMTVDKSTSTVYMELSSLRSEDTAVYYCARPPRAYGNYAGYWGQGTTVTVSSGGGGSSGAPRFLTRPKASVVSVGKDATLSCQIVGNPFPQVSWEKDKQPVTAGVRFRLAQDGDLYRLKILDLQLSDSGQYVCRARNAHGEAFACLGLQVDAEADKTHTCPPCPAPEAAGGPSVFLFPPKPKDTLMISRTPEVTCVVVDVSHEDPEVKFNWYVDGVEVHNAKTKPREEQYNSTYRVVSVLTVLHQDWLNGKEYKCKVSNKALPAPIEKTISKAKGQPREPQVCTLPPSREEMTKNQVSLSCAVKGFYPSDIAVEWESNGQPENNYKTTPPVLDSDGSFFLVSKLTVDKSRWQQGNVFSCSVMHEALHNHYTQKSLSLSPGK

SEQ ID NO: 107 - protein, 215 aa, synthetic construct
  CHAIN 1..215: note = P3-C7 L7H1-2-4
DVVMTQTPLSLPVTPGEPASISCRSSQSLVHSNQNTYLHWYLQKPGQSPQLLIYKVSNRFSGVPDRFSGSGSRTDFTLKISRVEAEDVGVYYCSQSTHVPYTFGGGTKVEIKGGGGSGIPPKIECLPIDISIDEGKVLTVASAFTGEPTPEVTWSTGGRKIHSQEQGRFHIENTDDSTTLTIKDVQKQDGGLYTLTLRNEFGSDSATVNIHIRSI

SEQ ID NO: 108 - protein, 447 aa, synthetic construct
  CHAIN 1..447: note = M81-2-3
EFQLQQSGPELVKPGASVKISCKASGYSFTDHNMNWVKQSNGKSLEWIGVMNPKFGTINYNQKFKDKATLTVDQSSSTAYMQLNSLTSEDSAVYYCVRDDYPNYFDYWGQGTTLTVSSGGGGSSGAPRFLTRPKASVVSVGKDATLSCQIVGNPFPQVSWEKDKQPVTAGVRFRLAQDGDLYRLKILDLQLSDSGQYVCRARNAHGEAFACLGLQVDAEADKTHTCPPCPAPEAAGGPSVFLFPPKPKDTLMISRTPEVTCVVVDVSHEDPEVKFNWYVDGVEVHNAKTKPREEQYNSTYRVVSVLTVLHQDWLNGKEYKCKVSNKALPAPIEKTISKAKGQPREPQVCTLPPSREEMTKNQVSLSCAVKGFYPSDIAVEWESNGQPENNYKTTPPVLDSDGSFFLVSKLTVDKSRWQQGNVFSCSVMHEALHNHYTQKSLSLSPGK

SEQ ID NO: 109 - protein, 209 aa, synthetic construct
  CHAIN 1..209: note = M81-2-4
QIVLTQSPAIMSASPGEKVTISCSASSSVNYMYWYQQKPGSSPKSWIYRTSNLASGVSARFSGSGSGTSYSLTISSMEAEDAATYYCQQYHDYPPTFGGGTKLEIKGGGGSGIPPKIECLPIDISIDEGKVLTVASAFTGEPTPEVTWSTGGRKIHSQEQGRFHIENTDDSTTLTIKDVQKQDGGLYTLTLRNEFGSDSATVNIHIRSI

SEQ ID NO: 110 - protein, 447 aa, synthetic construct
  CHAIN 1..447: note = 81 L1H1-2-3
EVQLVQSGAEVKKPGASVKVSCKASGYTFTDHNMNWVKQAPGQRLEWMGVMNPKFGTINYNQKFKDKATITRDTSASTAYMELSSLRSEDTAVYYCARDNYPNYFDYWGQGTTVTVSSGGGGSSGAPRFLTRPKASVVSVGKDATLSCQIVGNPFPQVSWEKDKQPVTAGVRFRLAQDGDLYRLKILDLQLSDSGQYVCRARNAHGEAFACLGLQVDAEADKTHTCPPCPAPEAAGGPSVFLFPPKPKDTLMISRTPEVTCVVVDVSHEDPEVKFNWYVDGVEVHNAKTKPREEQYNSTYRVVSVLTVLHQDWLNGKEYKCKVSNKALPAPIEKTISKAKGQPREPQVCTLPPSREEMTKNQVSLSCAVKGFYPSDIAVEWESNGQPENNYKTTPPVLDSDGSFFLVSKLTVDKSRWQQGNVFSCSVMHEALHNHYTQKSLSLSPGK

SEQ ID NO: 111 - protein, 209 aa, synthetic construct
  CHAIN 1..209: note = 81 L1H1-2-4
EIVLTQSPATLSLSPGERATLSCSASSSVNYMYWYQQKPGQAPKSWIYRTSNLASGVPARFSGSGSGTDYTLTISSLEPEDFAVYYCQQYHDYPPTFGGGTKVEIKGGGGSGIPPKIECLPIDISIDEGKVLTVASAFTGEPTPEVTWSTGGRKIHSQEQGRFHIENTDDSTTLTIKDVQKQDGGLYTLTLRNEFGSDSATVNIHIRSI

SEQ ID NO: 112 - protein, 209 aa, synthetic construct
  CHAIN 1..209: note = 81 L2H1-2-4
EIVLTQSPDFQSVTPGEKVTITCSASSSVNYMYWYQQKPDQSPKSWIYRTSNLASGVPSRFSGSGSGTDFTLTISSLEAEDAATYYCQQYHDYPPTFGGGTKVEIKGGGGSGIPPKIECLPIDISIDEGKVLTVASAFTGEPTPEVTWSTGGRKIHSQEQGRFHIENTDDSTTLTIKDVQKQDGGLYTLTLRNEFGSDSATVNIHIRSI

SEQ ID NO: 113 - protein, 209 aa, synthetic construct
  CHAIN 1..209: note = 81 L3H1-2-4
DIQLTQSPSFLSASPGDRVTITCSASSSVNYMYWYQQKPGSSPKSWIYRTSNLASGVPSRFSGSGSGTEYTLTISSLQPEDFATYYCQQYHDYPPTFGGGTKVEIKGGGGSGIPPKIECLPIDISIDEGKVLTVASAFTGEPTPEVTWSTGGRKIHSQEQGRFHIENTDDSTTLTIKDVQKQDGGLYTLTLRNEFGSDSATVNIHIRSI

SEQ ID NO: 114 - protein, 209 aa, synthetic construct
  CHAIN 1..209: note = 81 L4H1-2-4
DIQLTQSPSFLSASPGDRVTITCSASSSVNYMYWYQQKPGSSPKSWIYRTSNDASGVPSRFSGSGSGTEYTLTISSLQPEDFATYYCQQYHDYPPTFGGGTKVEIKGGGGSGIPPKIECLPIDISIDEGKVLTVASAFTGEPTPEVTWSTGGRKIHSQEQGRFHIENTDDSTTLTIKDVQKQDGGLYTLTLRNEFGSDSATVNIHIRSI

SEQ ID NO: 115 - protein, 209 aa, synthetic construct
  CHAIN 1..209: note = 81 L5H1-2-4
DIQLTQSPSFLSASPGDRVTITCSASSSVNYMYWYQQKPGSSPKSWIYRTSNLAQGVPSRFSGSGSGTEYTLTISSLQPEDFATYYCQQYHDYPPTFGGGTKVEIKGGGGSGIPPKIECLPIDISIDEGKVLTVASAFTGEPTPEVTWSTGGRKIHSQEQGRFHIENTDDSTTLTIKDVQKQDGGLYTLTLRNEFGSDSATVNIHIRSI

SEQ ID NO: 116 - protein, 209 aa, synthetic construct
  CHAIN 1..209: note = 81 L6H1-2-4
DIQLTQSPSFLSASPGDRVTITCSASSSVNYMYWYQQKPGSSPKSWIYRTQNLASGVPSRFSGSGSGTEYTLTISSLQPEDFATYYCQQYHDYPPTFGGGTKVEIKGGGGSGIPPKIECLPIDISIDEGKVLTVASAFTGEPTPEVTWSTGGRKIHSQEQGRFHIENTDDSTTLTIKDVQKQDGGLYTLTLRNEFGSDSATVNIHIRSI

SEQ ID NO: 117 - protein, 447 aa, synthetic construct
  CHAIN 1..447: note = M146-2-3
EFQLQQSGPELVKPGASVKISCKASGYSFTDYNMNWVKQSNGKSLEWIGLINPKYGTTNYNQKFKGKATLTVDQSSSTAYMQLNSLTSEDSAVYYCAIDDYPAWFAYWGQGTLVTVSAGGGGSSGAPRFLTRPKASVVSVGKDATLSCQIVGNPFPQVSWEKDKQPVTAGVRFRLAQDGDLYRLKILDLQLSDSGQYVCRARNAHGEAFACLGLQVDAEADKTHTCPPCPAPEAAGGPSVFLFPPKPKDTLMISRTPEVTCVVVDVSHEDPEVKFNWYVDGVEVHNAKTKPREEQYNSTYRVVSVLTVLHQDWLNGKEYKCKVSNKALPAPIEKTISKAKGQPREPQVCTLPPSREEMTKNQVSLSCAVKGFYPSDIAVEWESNGQPENNYKTTPPVLDSDGSFFLVSKLTVDKSRWQQGNVFSCSVMHEALHNHYTQKSLSLSPGK

SEQ ID NO: 118 - protein, 209 aa, synthetic construct
  CHAIN 1..209: note = M146-2-4
QIVLTQSPAIMSASPGEKVTISCSASSSLNYMYWYQQKPGSSPKSWIYRTSNLASGVPARFSGSGSGTSYSLTISSMEAEDAATYYCQQYHSYPPTFGAGTKLELKGGGGSGIPPKIECLPIDISIDEGKVLTVASAFTGEPTPEVTWSTGGRKIHSQEQGRFHIENTDDSTTLTIKDVQKQDGGLYTLTLRNEFGSDSATVNIHIRSI

SEQ ID NO: 119 - protein, 447 aa, synthetic construct
  CHAIN 1..447: note = 146 L1H1-2-3
EFQLVQSGAEVKKPGASVKVSCKASGYSFTDYNMNWVRQAPGQRLEWMGLINPKYGTTNYNQKFKGRVTLTVDQSSSTAYMELSSLRSEDTAVYYCARDNYPAWFAYWGQGTTVTVSSGGGGSSGAPRFLTRPKASVVSVGKDATLSCQIVGNPFPQVSWEKDKQPVTAGVRFRLAQDGDLYRLKILDLQLSDSGQYVCRARNAHGEAFACLGLQVDAEADKTHTCPPCPAPEAAGGPSVFLFPPKPKDTLMISRTPEVTCVVVDVSHEDPEVKFNWYVDGVEVHNAKTKPREEQYNSTYRVVSVLTVLHQDWLNGKEYKCKVSNKALPAPIEKTISKAKGQPREPQVCTLPPSREEMTKNQVSLSCAVKGFYPSDIAVEWESNGQPENNYKTTPPVLDSDGSFFLVSKLTVDKSRWQQGNVFSCSVMHEALHNHYTQKSLSLSPGK

SEQ ID NO: 120 - protein, 209 aa, synthetic construct
  CHAIN 1..209: note = 146 L1H1-2-4
EIVLTQSPATLSLSPGERATLSCSASSSLNYMYWYQQKPGSSPRPWIYRTSQLASGVPARFSGSGSGTDYTLTISSLEPEDFAVYYCQQYHSYPPTFGGGTKVEIKGGGGSGIPPKIECLPIDISIDEGKVLTVASAFTGEPTPEVTWSTGGRKIHSQEQGRFHIENTDDSTTLTIKDVQKQDGGLYTLTLRNEFGSDSATVNIHIRSI

SEQ ID NO: 121 - protein, 449 aa, synthetic construct
  CHAIN 1..449: note = P3-C7 L7H1-3-1
EVQLVQSGAEVKKPGASVKVSCKASGYTFTDHYIHWVRQAPGQGLEWMGVINPYNDGATYNQKFKGRVTMTVDKSTSTVYMELSSLRSEDTAVYYCARPPRAYGNYAGYWGQGTTVTVSSGGGGSSGAPRFLTRPKASVVSVGKDATLSCQIVGNPFPQVSWEKDKQPVTAGVRFRLAQDGDLYRLKILDLQLSDSGQYVCRARNAHGEAFACLGLQVDAEADKTHTCPPCPAPEAAGGPSVFLFPPKPKDTLMISRTPEVTCVVVDVSHEDPEVKFNWYVDGVEVHNAKTKPREEQYNSTYRVVSVLTVLHQDWLNGKEYKCKVSNKALPAPIEKTISKAKGQPREPQVYTLPPCREEMTKNQVSLWCLVKGFYPSDIAVEWESNGQPENNYKTTPPVLDSDGSFFLYSKLTVDKSRWQQGNVFSCSVMHEALHNHYTQKSLSLSPGK

SEQ ID NO: 122 - protein, 447 aa, synthetic construct
  DOMAIN 1..447: note = 81 L1H1-3-1
EVQLVQSGAEVKKPGASVKVSCKASGYTFTDHNMNWVKQAPGQRLEWMGVMNPKFGTINYNQKFKDKATITRDTSASTAYMELSSLRSEDTAVYYCARDNYPNYFDYWGQGTTVTVSSGGGGSSGAPRFLTRPKASVVSVGKDATLSCQIVGNPFPQVSWEKDKQPVTAGVRFRLAQDGDLYRLKILDLQLSDSGQYVCRARNAHGEAFACLGLQVDAEADKTHTCPPCPAPEAAGGPSVFLFPPKPKDTLMISRTPEVTCVVVDVSHEDPEVKFNWYVDGVEVHNAKTKPREEQYNSTYRVVSVLTVLHQDWLNGKEYKCKVSNKALPAPIEKTISKAKGQPREPQVYTLPPCREEMTKNQVSLWCLVKGFYPSDIAVEWESNGQPENNYKTTPPVLDSDGSFFLYSKLTVDKSRWQQGNVFSCSVMHEALHNHYTQKSLSLSPGK

SEQ ID NO: 123 - protein, 447 aa, synthetic construct
  CHAIN 1..447: note = 146 L1H1-3-1
EFQLVQSGAEVKKPGASVKVSCKASGYSFTDYNMNWVRQAPGQRLEWMGLINPKYGTTNYNQKFKGRVTLTVDQSSSTAYMELSSLRSEDTAVYYCARDNYPAWFAYWGQGTTVTVSSGGGGSSGAPRFLTRPKASVVSVGKDATLSCQIVGNPFPQVSWEKDKQPVTAGVRFRLAQDGDLYRLKILDLQLSDSGQYVCRARNAHGEAFACLGLQVDAEADKTHTCPPCPAPEAAGGPSVFLFPPKPKDTLMISRTPEVTCVVVDVSHEDPEVKFNWYVDGVEVHNAKTKPREEQYNSTYRVVSVLTVLHQDWLNGKEYKCKVSNKALPAPIEKTISKAKGQPREPQVYTLPPCREEMTKNQVSLWCLVKGFYPSDIAVEWESNGQPENNYKTTPPVLDSDGSFFLYSKLTVDKSRWQQGNVFSCSVMHEALHNHYTQKSLSLSPGK

SEQ ID NO: 124 - protein, 702 aa, synthetic construct
  CHAIN 1..702: note = P3-C7 L7H1-4-1
EVQLVQSGAEVKKPGASVKVSCKASGYTFTDHYIHWVRQAPGQGLEWMGVINPYNDGATYNQKFKGRVTMTVDKSTSTVYMELSSLRSEDTAVYYCARPPRAYGNYAGYWGQGTTVTVSSASTKGPSVFPLAPSSKSTSGGTAALGCLVKDYFPEPVTVSWNSGALTSGVHTFPAVLQSSGLYSLSSVVTVPSSSLGTQTYICNVNHKPSNTKVDKKVEPKSCEVQLVESGGGLVQPGGSLKLSCAASGFTFNKYAMNWVRQAPGKGLEWVARIRSKYNNYATYYADSVKDRFTISRDDSKNTAYLQMNNLKTEDTAVYYCVRHGNFGNEYISYWAYWGQGTLVTVSSGGGGSGGGGSGGGGSQTVVTQEPSLTVSPGGTVTLTCGSSTGAVTSGNYPNWVQQKPGQAPRGLIGGTKFLAPGTPARFSGSLLGGKAALTLSGVQPEDEAEYYCVLWYSNRWVFGGGTKLTVLGGGDKTHTCPPCPAPEAAGGPSVFLFPPKPKDTLMISRTPEVTCVVVDVSHEDPEVKFNWYVDGVEVHNAKTKPREEQYNSTYRVVSVLTVLHQDWLNGKEYKCKVSNKALPAPIEKTISKAKGQPREPQVYTLPPSREEMTKNQVSLTCLVKGFYPSDIAVEWESNGQPENNYKTTPPVLDSDGSFFLYSKLTVDKSRWQQGNVFSCSVMHEALHNHYTQKSLSLSPGK

SEQ ID NO: 125 - protein, 687 aa, synthetic construct
  CHAIN 1..687: note = P3-C7 L7H1-5-1
EVQLVQSGAEVKKPGASVKVSCKASGYTFTDHYIHWVRQAPGQGLEWMGVINPYNDGATYNQKFKGRVTMTVDKSTSTVYMELSSLRSEDTAVYYCARPPRAYGNYAGYWGQGTTVTVSSASTKGPSVFPLAPSSKSTSGGTAALGCLVKDYFPEPVTVSWNSGALTSGVHTFPAVLQSSGLYSLSSVVTVPSSSLGTQTYICNVNHKPSNTKVDKKVEPKSCGGGGSGGGGSEVQLVESGGGLVQPGGSLKLSCAASGFTFNKYAMNWVRQAPGKGLEWVARIRSKYNNYATYYADSVKDRFTISRDDSKNTAYLQMNNLKTEDTAVYYCVRHGNFGNEYISYWAYWGQGTLVTVSSGGGGSSGAPRFLTRPKASVVSVGKDATLSCQIVGNPFPQVSWEKDKQPVTAGVRFRLAQDGDLYRLKILDLQLSDSGQYVCRARNAHGEAFACLGLQVDAEADKTHTCPPCPAPEAAGGPSVFLFPPKPKDTLMISRTPEVTCVVVDVSHEDPEVKFNWYVDGVEVHNAKTKPREEQYNSTYRVVSVLTVLHQDWLNGKEYKCKVSNKALPAPIEKTISKAKGQPREPQVYTLPPSREEMTKNQVSLTCLVKGFYPSDIAVEWESNGQPENNYKTTPPVLDSDGSFFLYSKLTVDKSRWQQGNVFSCSVMHEALHNHYTQKSLSLSPGK

SEQ ID NO: 126 - protein, 461 aa, synthetic construct
  CHAIN 1..461: note = GUCY2c-1608 -Knob
DIQLTQSPSSLSASVGDRVTITCRASESVDYYGSSLLQWYQQKPGKAPKLLIYAASKLASGVPSRFSGSGSGTDFTLTISSLQPEDFATYYCQQTRKAYTFGQGTKLEIKGGGSGGGGEVQLVESGGGLVQPGGSLRLSCAASGFTFSDYYMTWVRQAPGKGLEWVAFIRNQARGYTSDHNPSVKGRFTISRDNAKNSLYLQMNSLRAEDTAVYYCARDRPSYYVLDYWGQGTTVTVSSGCPPCPAPEAAGAPSVFLFPPKPKDTLMISRTPEVTCVVVDVSHEDPEVKFNWYVDGVEVHNAKTKPREEQYNSTYRVVSVLTVLHQDWLNGKEYKCKVSNKALPAPIEKTISKAKGQPREPQVCTLPPSREEMTKNQVSLWCLVKGFYPSDIAVEWESNGQPENNYKTTPPVLDSDGSFFLYSKLTVDKSRWQQGNVFSCSVMHEALHNHYTQKSLSLSPG

SEQ ID NO: 127 - protein, 465 aa, synthetic construct
  CHAIN 1..465: note = GUCY2c-1608 -Hole
DIQMTQSPSSLSASVGDRVTITCTSSQSLFNVRSQKNYLAWYQQKPGKAPKLLIYWASTRESGVPSRFSGSGSGTDFTLTISSLQPEDFATYYCKQSYDLFTFGGGTKVEIKGGGGSGGGGEVQLVESGGGLVQPGGSLRLSCAASGFTFSSYWMHWVRQAPGKGLEWIGEIKPSNELTNVHEKFKDRFTISVDKAKNSAYLQMNSLRAEDTAVYYCTRTITTTEGYWFFDVWGQGTLVTVSSGCPPCPAPEAAGAPSVFLFPPKPKDTLMISRTPEVTCVVVDVSHEDPEVKFNWYVDGVEVHNAKTKPREEQYNSTYRVVSVLTVLHQDWLNGKEYKCKVSNKALPAPIEKTISKAKGQPREPQVYTLPPCREEMTKNQVSLSCAVKGFYPSDIAVEWESNGQPENNYKTTPPVLDSDGSFFLVSKLTVDKSRWQQGNVFSCSVMHEALHNHYTQKSLSLSPG

SEQ ID NO: 128 - protein, 5 aa, synthetic construct
  DOMAIN 1..5: note = GUCY2C-HCDR1
SYWMH

SEQ ID NO: 129 - protein, 17 aa, synthetic construct
  DOMAIN 1..17: note = GUCY2C-HCDR2
EIKPSNELTNVHEKFKD

SEQ ID NO: 130 - protein, 13 aa, synthetic construct
  DOMAIN 1..13: note = GUCY2C-HCDR3
TITTTEGYWFFDV

SEQ ID NO: 131 - protein, 15 aa, synthetic construct
  DOMAIN 1..15: note = GUCY2C-LCDR1
RASESVDYYGSSLLQ

SEQ ID NO: 132 - protein, 7 aa, synthetic construct
  DOMAIN 1..7: note = GUCY2C-LCDR2
AASKLAS

SEQ ID NO: 133 - protein, 8 aa, synthetic construct
  DOMAIN 1..8: note = GUCY2C-LCDR3
QQTRKAYT

SEQ ID NO: 134 - protein, 5 aa, synthetic construct
  DOMAIN 1..5: note = CD3-HCDR1
DYYMT

SEQ ID NO: 135 - protein, 19 aa, synthetic construct
  DOMAIN 1..19: note = CD3-HCDR2
FIRNQARGYTSDHNPSVKG

SEQ ID NO: 136 - protein, 10 aa, synthetic construct
  DOMAIN 1..10: note = CD3-HCDR3
DRPSYYVLDY

SEQ ID NO: 137 - protein, 17 aa, synthetic construct
  DOMAIN 1..17: note = CD3-LCDR1
TSSQSLFNVRSQKNYLA

SEQ ID NO: 138 - protein, 7 aa, synthetic construct
  DOMAIN 1..7: note = CD3-LCDR2
WASTRES

SEQ ID NO: 139 - protein, 8 aa, synthetic construct
  DOMAIN 1..8: note = CD3-LCDR3
KQSYDLFT

SEQ ID NO: 140 - protein, 5 aa, synthetic construct
  DOMAIN 1..5: note = EGFR-HCDR1
TYGMH

SEQ ID NO: 141 - protein, 17 aa, synthetic construct
  DOMAIN 1..17: note = EGFR-HCDR2
VIWDDGSYKYYGDSVKG

SEQ ID NO: 142 - protein, 16 aa, synthetic construct
  DOMAIN 1..16: note = EGFR-HCDR3
DGITMVRGVMKDYFDY

SEQ ID NO: 143 - protein, 11 aa, synthetic construct
  DOMAIN 1..11: note = EGFR-LCDR1
RASQDISSALV

SEQ ID NO: 144 - protein, 7 aa, synthetic construct
  DOMAIN 1..7: note = EGFR-LCDR2
DASSLES

SEQ ID NO: 145 - protein, 9 aa, synthetic construct
  DOMAIN 1..9: note = EGFR-LCDR3
QQFNSYPLT

SEQ ID NO: 146 - protein, 5 aa, synthetic construct
  DOMAIN 1..5: note = CD28-HCDR1
SYWIT

SEQ ID NO: 147 - protein, 17 aa, synthetic construct
  DOMAIN 1..17: note = CD28-HCDR2
DIYPGSGRTNYNEMFKN

SEQ ID NO: 148 - protein, 12 aa, synthetic construct
  DOMAIN 1..12: note = CD28-HCDR3
RHYGTGYESFDV

SEQ ID NO: 149 - protein, 11 aa, synthetic construct
  DOMAIN 1..11: note = CD28-LCDR1
RASQDISNYLN

SEQ ID NO: 150 - protein, 7 aa, synthetic construct
  DOMAIN 1..7: note = CD28-LCDR2
YTSRLHS

SEQ ID NO: 151 - protein, 9 aa, synthetic construct
  DOMAIN 1..9: note = CD28-LCDR3
QQGNTLPWT

SEQ ID NO: 152 - protein, 125 aa, synthetic construct [sequence omitted]

SEQ ID NO: 153 - protein, 107 aa, synthetic construct
  DOMAIN 1..107: note = EGFR-VL
DIQLTQSPSSLSASVGDRVTITCRASQDISSALVWYQQKPGKAPKLLIYDASSLESGVPSRFSGSESGTDFTLTISSLQPEDFATYYCQQFNSYPLTFGGGTKVEIK

SEQ ID NO: 154 - protein, 121 aa, synthetic construct
  DOMAIN 1..121: note = CD28-VH
EVQLVQSGAEVKKPGASVKVSCKASGYTLTSYWITWVRQAPGQGLEWMGDIYPGSGRTNYNEMFKNRVTMTVDTSTSTAYMELSSLRSEDTAVYYCARRHYGTGYESFDVWGQGTTVTVSS

SEQ ID NO: 155 - protein, 107 aa, synthetic construct
  DOMAIN 1..107: note = CD28-VL
DIQMTQSPSSLSASVGDRVTITCRASQDISNYLNWYQQKPDGTIKLLIYYTSRLHSGVPSRFSGSGSGTDYTFTISSLQPEDIATYYCQQGNTLPWTFGGGTKVEIK

SEQ ID NO: 156 - protein, 451 aa, synthetic construct
  CHAIN 1..451: note = 97H2L3OT-ZAL-1
EVQLVQSGAEVKKPGASVKVSCKASGYTLTSYWITWVRQAPGQGLEWMGDIYPGSGRTNYNEMFKNRVTMTVDTSTSTAYMELSSLRSEDTAVYYCARRHYGTGYESFDVWGQGTTVTVSSGGGGSGIPPKIECLPIDISIDEGKVLTVASAFTGEPTPEVTWSTGGRKIHSQEQGRFHIENTDDSTTLTIKDVQKQDGGLYTLTLRNEFGSDSATVNIHIRSIDKTHTCPPCPAPEAAGGPSVFLFPPKPKDTLMISRTPEVTCVVVDVSHEDPEVKFNWYVDGVEVHNAKTKPREEQYNSTYRVVSVLTVLHQDWLNGKEYKCKVSNKALPAPIEKTISKAKGQPREPQVYTLPPCRDELTKNQVSLWCLVKGFYPSDIAVEWESNGQPENNYKTTPPVLDSDGSFFLYSKLTVDKSRWQQGNVFSCSVMHEALHNHYTQKSLSLSPGK

SEQ ID NO: 157 - protein, 209 aa, synthetic construct
  CHAIN 1..209: note = 97H2L3OT-ZAL-2
DIQMTQSPSSLSASVGDRVTITCRASQDISNYLNWYQQKPDGTIKLLIYYTSRLHSGVPSRFSGSGSGTDYTFTISSLQPEDIATYYCQQGNTLPWTFGGGTKVEIKGGGGSSGAPRFLTRPKASVVSVGKDATLSCQIVGNPFPQVSWEKDKQPVTAGVRFRLAQDGDLYRLKILDLQLSDSGQYVCRARNAHGEAFACLGLQVDAEA

SEQ ID NO: 158 - protein, 455 aa, synthetic construct
  CHAIN 1..455: note = 97H2L3OT-ZAL-3
QVQLVESGGGVVQPGRSLRLSCAASGFTFSTYGMHWVRQAPGKGLEWVAVIWDDGSYKYYGDSVKGRFTISRDNSKNTLYLQMNSLRAEDTAVYYCARDGITMVRGVMKDYFDYWGQGTLVTVSSASTKGPSVFPLAPSSKSTSGGTAALGCLVKDYFPEPVTVSWNSGALTSGVHTFPAVLQSSGLYSLSSVVTVPSSSLGTQTYICNVNHKPSNTKVDKKVEPKSCDKTHTCPPCPAPEAAGGPSVFLFPPKPKDTLMISRTPEVTCVVVDVSHEDPEVKFNWYVDGVEVHNAKTKPREEQYNSTYRVVSVLTVLHQDWLNGKEYKCKVSNKALPAPIEKTISKAKGQPREPQVCTLPPSRDELTKNQVSLSCAVKGFYPSDIAVEWESNGQPENNYKTTPPVLDSDGSFFLVSKLTVDKSRWQQGNVFSCSVMHEALHNHYTQKSLSLSPGK

SEQ ID NO: 159 - protein, 214 aa, synthetic construct
  CHAIN 1..214: note = 97H2L3OT-ZAL-4
DIQLTQSPSSLSASVGDRVTITCRASQDISSALVWYQQKPGKAPKLLIYDASSLESGVPSRFSGSESGTDFTLTISSLQPEDFATYYCQQFNSYPLTFGGGTKVEIKRTVAAPSVFIFPPSDEQLKSGTASVVCLLNNFYPREAKVQWKVDNALQSGNSQESVTEQDSKDSTYSLSSTLTLSKADYEKHKVYACEVTHQGLSSPVTKSFNRGEC

SEQ ID NO: 160 - protein, 5 aa, synthetic construct
  DOMAIN 1..5: note = CD28-HCDR1
SHWIQ

SEQ ID NO: 161 - protein, 17 aa, synthetic construct
  DOMAIN 1..17: note = CD28-HCDR2
EIFPGSGSTHYNEKFKG

SEQ ID NO: 162 - protein, 12 aa, synthetic construct
  DOMAIN 1..12: note = CD28-HCDR3
LHYGTSYDAMDY

SEQ ID NO: 163 - protein, 9 aa, synthetic construct
  DOMAIN 1..9: note = CD28-LCDR3
QQGYTLPRT

SEQ ID NO: 164 - protein, 121 aa, synthetic construct
  DOMAIN 1..121: note = CD28-VH
EVQLVQSGAEVKKPGASVKVSCKAPGYTFTSHWIQWVRQAPGQGLEWMGEIFPGSGSTHYNEKFKGRVTMTVDTSTSTAYMELSSLRSEDTAVYYCARLHYGTSYDAMDYWGQGTTVTVSS

SEQ ID NO: 165 - protein, 107 aa, synthetic construct
  DOMAIN 1..107: note = CD28-VL
DIQMTQSPSSLSASVGDRVTITCRASQDISNYLNWYQQKPGKAVKLLIYYTSRLHSGVPSRFSGSGSGTDFTFTISSLQPEDIATYYCQQGYTLPRTFGGGTKVEIK

SEQ ID NO: 166 - protein, 451 aa, synthetic construct
  CHAIN 1..451: note = 129H4L1OT-ZAL-1
EVQLVQSGAEVKKPGASVKVSCKAPGYTFTSHWIQWVRQAPGQGLEWMGEIFPGSGSTHYNEKFKGRVTMTVDTSTSTAYMELSSLRSEDTAVYYCARLHYGTSYDAMDYWGQGTTVTVSSGGGGSGIPPKIECLPIDISIDEGKVLTVASAFTGEPTPEVTWSTGGRKIHSQEQGRFHIENTDDSTTLTIKDVQKQDGGLYTLTLRNEFGSDSATVNIHIRSIDKTHTCPPCPAPEAAGGPSVFLFPPKPKDTLMISRTPEVTCVVVDVSHEDPEVKFNWYVDGVEVHNAKTKPREEQYNSTYRVVSVLTVLHQDWLNGKEYKCKVSNKALPAPIEKTISKAKGQPREPQVYTLPPCRDELTKNQVSLWCLVKGFYPSDIAVEWESNGQPENNYKTTPPVLDSDGSFFLYSKLTVDKSRWQQGNVFSCSVMHEALHNHYTQKSLSLSPGK

SEQ ID NO: 167 - protein, 209 aa, synthetic construct
  CHAIN 1..209: note = 129H4L1OT-ZAL-2
DIQMTQSPSSLSASVGDRVTITCRASQDISNYLNWYQQKPGKAVKLLIYYTSRLHSGVPSRFSGSGSGTDFTFTISSLQPEDIATYYCQQGYTLPRTFGGGTKVEIKGGGGSSGAPRFLTRPKASVVSVGKDATLSCQIVGNPFPQVSWEKDKQPVTAGVRFRLAQDGDLYRLKILDLQLSDSGQYVCRARNAHGEAFACLGLQVDAEA

SEQ ID NO: 168 - protein, 5 aa, synthetic construct
  DOMAIN 1..5: note = CD28-HCDR1
GYYMN

SEQ ID NO: 169 - protein, 17 aa, synthetic construct
  DOMAIN 1..17: note = CD28-HCDR2
EINPSTGDTTYNQKFKA

SEQ ID NO: 170 - protein, 10 aa, synthetic construct
  DOMAIN 1..10: note = CD28-HCDR3
PYYDLTPFLY

SEQ ID NO: 171 - protein, 11 aa, synthetic construct
  DOMAIN 1..11: note = CD28-LCDR1
LASQTIGTWLA

SEQ ID NO: 172 - protein, 7 aa, synthetic construct
  DOMAIN 1..7: note = CD28-LCDR2
AATTGAD

SEQ ID NO: 173 - protein, 9 aa, synthetic construct
  DOMAIN 1..9: note = CD28-LCDR3
QQLYSTPYT

SEQ ID NO: 174 - protein, 119 aa, synthetic construct
  DOMAIN 1..119: note = CD28-VH
EVQLVQSGAEVKKPGASVKVSCKASGYSFTGYYMNWVRQAPGQRLEWMGEINPSTGDTTYNQKFKAKVTLTVDKSASTAYMELSSLRSEDTAVYYCASPYYDLTPFLYWGQGTLVTVSS

SEQ ID NO: 175 - protein, 107 aa, synthetic construct
  DOMAIN 1..107: note = CD28-VL
DIQMTQSPSSVSASVGDRVTITCLASQTIGTWLAWYQQKPGKSPKLLIYAATTGADGVPSRFSGSGSGTKFTLTISSLQPEDFATYYCQQLYSTPYTFGGGTKVEIK

SEQ ID NO: 176 - protein, 449 aa, synthetic construct
  CHAIN 1..449: note = 94H6L12-ZALOT-1
EVQLVQSGAEVKKPGASVKVSCKASGYSFTGYYMNWVRQAPGQRLEWMGEINPSTGDTTYNQKFKAKVTLTVDKSASTAYMELSSLRSEDTAVYYCASPYYDLTPFLYWGQGTLVTVSSASTKGPSVFPLAPSSKSTSGGTAALGCLVKDYFPEPVTVSWNSGALTSGVHTFPAVLQSSGLYSLSSVVTVPSSSLGTQTYICNVNHKPSNTKVDKKVEPKSCDKTHTCPPCPAPEAAGGPSVFLFPPKPKDTLMISRTPEVTCVVVDVSHEDPEVKFNWYVDGVEVHNAKTKPREEQYNSTYRVVSVLTVLHQDWLNGKEYKCKVSNKALPAPIEKTISKAKGQPREPQVYTLPPCRDELTKNQVSLWCLVKGFYPSDIAVEWESNGQPENNYKTTPPVLDSDGSFFLYSKLTVDKSRWQQGNVFSCSVMHEALHNHYTQKSLSLSPGK

SEQ ID NO: 177 - protein, 214 aa, synthetic construct
  DOMAIN 1..214: note = 94H6L12-ZALOT-2
DIQMTQSPSSVSASVGDRVTITCLASQTIGTWLAWYQQKPGKSPKLLIYAATTGADGVPSRFSGSGSGTKFTLTISSLQPEDFATYYCQQLYSTPYTFGGGTKVEIKRTVAAPSVFIFPPSDEQLKSGTASVVCLLNNFYPREAKVQWKVDNALQSGNSQESVTEQDSKDSTYSLSSTLTLSKADYEKHKVYACEVTHQGLSSPVTKSFNRGEC

SEQ ID NO: 178 - protein, 454 aa, synthetic construct
  DOMAIN 1..454: note = 94H6L12-ZALOT-3
QVQLVESGGGVVQPGRSLRLSCAASGFTFSTYGMHWVRQAPGKGLEWVAVIWDDGSYKYYGDSVKGRFTISRDNSKNTLYLQMNSLRAEDTAVYYCARDGITMVRGVMKDYFDYWGQGTLVTVSSGGGGSSGAPRFLTRPKASVVSVGKDATLSCQIVGNPFPQVSWEKDKQPVTAGVRFRLAQDGDLYRLKILDLQLSDSGQYVCRARNAHGEAFACLGLQVDAEADKTHTCPPCPAPEAAGGPSVFLFPPKPKDTLMISRTPEVTCVVVDVSHEDPEVKFNWYVDGVEVHNAKTKPREEQYNSTYRVVSVLTVLHQDWLNGKEYKCKVSNKALPAPIEKTISKAKGQPREPQVCTLPPSRDELTKNQVSLSCAVKGFYPSDIAVEWESNGQPENNYKTTPPVLDSDGSFFLVSKLTVDKSRWQQGNVFSCSVMHEALHNHYTQKSLSLSPGK

SEQ ID NO: 179 - protein, 210 aa, synthetic construct
  CHAIN 1..210: note = 94H6L12-ZALOT-4
DIQLTQSPSSLSASVGDRVTITCRASQDISSALVWYQQKPGKAPKLLIYDASSLESGVPSRFSGSESGTDFTLTISSLQPEDFATYYCQQFNSYPLTFGGGTKVEIKGGGGSGIPPKIECLPIDISIDEGKVLTVASAFTGEPTPEVTWSTGGRKIHSQEQGRFHIENTDDSTTLTIKDVQKQDGGLYTLTLRNEFGSDSATVNIHIRSI

SEQ ID NO: 180 - protein, 118 aa, synthetic construct
  DOMAIN 1..118: note = VH2-L
QVQLVESGGGVVQPGRSLRLSCAASGFTFSSYTMHWVRQAPGKGLEWVTFISYDGNNKYYADSVKGRFTISRDNSKNTLYLQMNSLRAEDTAIYYCARTGWLGPFDYWGQGTLVTVSS

SEQ ID NO: 181 - protein, 108 aa, synthetic construct
  DOMAIN 1..108: note = VH2-L
EIVLTQSPGTLSLSPGERATLSCRASQSVGSSYLAWYQQKPGQAPRLLIYGAFSRATGIPDRFSGSGSGTDFTLTISRLEPEDFAVYYCQQYGSSPWTFGQGTKVEIK

SEQ ID NO: 182 - protein, 98 aa, synthetic construct
  DOMAIN 1..98: note = T.0
GIPPKIEALPSDISIDEGKVLTVACAFTGEPTPEVTWSCGGRKIHSQEQGRFHIENTDDLTTLIIMDVQKQDGGLYTLSLGNEFGSDSATVNIHIRSI

SEQ ID NO: 183 - protein, 98 aa, synthetic construct
  DOMAIN 1..98: note = T.1
GIPPKIECLPSDISIDEGKVLTVASAFTGEPTPEVTWSTGGRKIHSQEQGRFHIENTDDLTTLIIMDVQKQDGGLYTLSLGNEFGSDSATVNIHIRSI

SEQ ID NO: 184 - protein, 98 aa, synthetic construct
  DOMAIN 1..98: note = T.2
GIPPKIEALPSDISIDEGKCLTVASAFTGEPTPEVTWSTGGRKIHSQEQGRFHIENTDDLTTLIIMDVQKQDGGLYTLSLGNEFGSDSATVNIHIRSI

SEQ ID NO: 185 - protein, 98 aa, synthetic construct
  DOMAIN 1..98: note = T.3
GIPPKIEALPSDISIDEGKVLTVASCFTGEPTPEVTWSTGGRKIHSQEQGRFHIENTDDLTTLIIMDVQKQDGGLYTLSLGNEFGSDSATVNIHIRSI

SEQ ID NO: 186 - protein, 98 aa, synthetic construct
  DOMAIN 1..98: note = T.4
GIPPKIEALPSDISIDEGKVLCVASAFTGEPTPEVTWSTGGRKIHSQEQGRFHIENTDDLTTLIIMDVQKQDGGLYTLSLGNEFGSDSATVNIHIRSI

SEQ ID NO: 187 - protein, 103 aa, synthetic construct
  DOMAIN 1..103: note = T.5
KAGIRGIPPKIECLPSDISIDEGKVLTVASAFTGEPTPEVTWSTGGRKIHSQEQGRFHIENTDDLTTLIIMDVQKQDGGLYTLSLGNEFGSDSATVNIHIRSI

SEQ ID NO: 188 - protein, 103 aa, synthetic construct
  DOMAIN 1..103: note = T.6
KAGIRGIPPKIEALPSDISIDEGKVLTVACAFTGEPTPEVTWSCGGRKIHSQEQGRFHIENTDDLTTLIIMDVQKQDGGLYTLSLGNEFGSDSATVNIHIRSI

SEQ ID NO: 189 - protein, 98 aa, synthetic construct
  DOMAIN 1..98: note = T.7
GIPPKIECLPSDISIDEGKVLTVASAFTGEPTPEVTWSTGGRKIHSQEQGRFHIENTDDLTTLIISDVQKQDGGLYSLSLGNEFGSDSATVNIHIRSI

SEQ ID NO: 190 - protein, 98 aa, synthetic construct
  DOMAIN 1..98: note = T.8
GIPPKIECLPSDISIDEGKVLTVASAFTGEPTPEVTWSTGGRKIHSQEQGRFHIENTDDLTTLIIKDVQRQDGGLYTLTLRNEFGSDSATVNIHIRSI

SEQ ID NO: 191 - protein, 98 aa, synthetic construct
  DOMAIN 1..98: note = T.9
GIWPKIECLPIDLSIDEGKVLMVASAFTGEPTPEVTWSTGGRKIHSQEQGRFHIENTDDLTTLIIMDVQKQDGGLYTLSLGMEFGSDSATVNIHIRSI

SEQ ID NO: 192 - protein, 98 aa, synthetic construct
  DOMAIN 1..98: note = T.10
GIPPKIECLPIDISIDEGKVLTVASAFTGEPTPEVTWSTGGRKIHSQEQGRFHIENTDDLTTLIIKDVQKQDGGLYTLTLRNEFGSDSATVNIHIRSI

SEQ ID NO: 193 - protein, 98 aa, synthetic construct
  DOMAIN 1..98: note = T.11
GIPPKIECLPSDISIDEGKVLTVASAFTGEPTPEVTWSTSGKKISSEEGGRFHIESTEDLTTLIIMDVQKQDGGVYTLSLGNDLGSDSATVNIHIRSI

SEQ ID NO: 194 - protein, 98 aa, synthetic construct
  DOMAIN 1..98: note = T.12
GIPPKIECLPSDISIDEGKVLTVASAFTGEPTPEVTWSTGGRKIHSEEGGRFHIESTEDLTTLIIMDVQKQDGGVYTLSLGNEFGSDSATVNIHIRSI

SEQ ID NO: 195 - protein, 98 aa, synthetic construct
  DOMAIN 1..98: note = T.13
GIPPKIECLPSDISIDEGKVLTVASAFTGEPTPEVTWSTGGRKIHSQEQGRFHIESTEDLTTLIIMDVQKQDGGVYTLSLGNEFGSDSATVNIHIRSI

SEQ ID NO: 196 - protein, 98 aa, synthetic construct
  DOMAIN 1..98: note = T.14
GIPPKIECLPSDISIDEGKVLTVASAFTGEPTPEVTWSTGGRKIHSQEQGRFHIESTEDLTTLIISDVQKQDGGLYSLSLGNEFGSDSATVNIHIRSI

SEQ ID NO: 197 - protein, 103 aa, synthetic construct
  DOMAIN 1..103: note = T.15
KAGIRGIPPKIECLPSDISIDEGKVLTVASAFTGEPTPEVTWSTGGRKIHSQEQGRFHIESTEDLTTLIISDVQKQDGGLYSLSLGNEFGSDSATVNIHIRSI

SEQ ID NO: 198 - protein, 98 aa, synthetic construct
  DOMAIN 1..98: note = T.16
GIPPKIECLPIDISIDEGKVLTVASAFTGEPTPEVTWSTGGRKIHSQEQGRFHIENTDDSTTLTIKDVQKQDGGLYTLTLRNEFGSDSATVNIHIRSI

SEQ ID NO: 199 - protein, 98 aa, synthetic construct
  DOMAIN 1..98: note = T.17
GIPPKIECLPIDISIDEGKCLTVASAFTGEPTPEVTWSTGGRKIHSQEQGRFHIENTDDSTTLTIKDVQKQDGGLYTLTLRNEFGSDSATVNIHIRSI

SEQ ID NO: 200 - protein, 98 aa, synthetic construct
  DOMAIN 1..98: note = T.18
GIPPKIECLPIDISIDEGKVLTVASCFTGEPTPEVTWSTGGRKIHSQEQGRFHIENTDDSTTLTIKDVQKQDGGLYTLTLRNEFGSDSATVNIHIRSI

SEQ ID NO: 201 - protein, 97 aa, synthetic construct
  DOMAIN 1..97: note = O.0
SGAPRFLTRPKAFVVSVGKDATLSCQIVGNPTPQVSWEKDQQPVAAGARFRLAQDGDLYRLTILDLALGDSGQYVCRARNAIGEAFAAVGLQVDAEA

SEQ ID NO: 202 - protein, 98 aa, synthetic construct
  DOMAIN 1..98: note = OL.0
QGSPPCFLRFPRPVRVVSGAEAELKCVVLGEPPPVVVWEKGGQQLAASERLSFPADGAEHGLLLTAALPTDAGVYVCRARNAAGEAYAAAAVTVLEPP

SEQ ID NO: 203 - protein, 97 aa, synthetic construct
  DOMAIN 1..97: note = O.1
SGAPRFLTRPKAFVVSVGKDATLSCQIVGNPTPQVSWEKDQQPVAAGARFRLAQDGDLYRLTILDLALGDSGQYVCRARNAIGEAFACVGLQVDAEA

SEQ ID NO: 204 - protein, 97 aa, synthetic construct
  DOMAIN 1..97: note = O.2
SGCPRFLTRPKAFVVSVGKDATLSCQIVGNPTPQVSWEKDQQPVAAGARFRLAQDGDLYRLTILDLALGDSGQYVCRARNAIGEAFAAVGLQVDAEA

SEQ ID NO: 205 - protein, 97 aa, synthetic construct
  DOMAIN 1..97: note = O.3
SGAPRFLTCPKAFVVSVGKDATLSCQIVGNPTPQVSWEKDQQPVAAGARFRLAQDGDLYRLTILDLALGDSGQYVCRARNAIGEAFAAVGLQVDAEA

SEQ ID NO: 206 - protein, 97 aa, synthetic construct
  DOMAIN 1..97: note = O.4
SGAPRFLTRPKAFVVSVGKDATLSSQIVGNPTPQVSWEKDQQPVAAGARFRLAQDGDLYRLTILDLALGDSGQYVSRARNAIGEAFACVGLQVDAEA

SEQ ID NO: 207 - protein, 97 aa, synthetic construct
  DOMAIN 1..97: note = O.5
SGCPRFLTRPKAFVVSVGKDATLSSQIVGNPTPQVSWEKDQQPVAAGARFRLAQDGDLYRLTILDLALGDSGQYVSRARNAIGEAFAAVGLQVDAEA

SEQ ID NO: 208 - protein, 97 aa, synthetic construct
  DOMAIN 1..97: note = O.6
SGAPRFLTCPKAFVVSVGKDATLSSQIVGNPTPQVSWEKDQQPVAAGARFRLAQDGDLYRLTILDLALGDSGQYVSRARNAIGEAFAAVGLQVDAEA

SEQ ID NO: 209 - protein, 97 aa, synthetic construct
  DOMAIN 1..97: note = O.7
SGAPRFKTRPKAFVVSVGKDATLSSQIVGNPTPQVSWEKDQQPVAAGARFRLAQDGDLYRLKILDLALGDSGQYVSRARNAIGEAFACVGLQVDAEA

SEQ ID NO: 210 - protein, 97 aa, synthetic construct
  DOMAIN 1..97: note = O.8
SGAPRFKTRPKAFVVSVGKDATLSSQIVGNPTPQVSWEKDQQPVAAGARFRLAQDGDLYRLHILDLALGDSGQYVSRARNAIGEAFACVGLQVDAEA

SEQ ID NO: 211 - protein, 97 aa, synthetic construct
  DOMAIN 1..97: note = O.9
SGAPRFLTRPLAFVVSVGKDATLSSQIVGNPTPQVSWEKDQQPVAAGARFRLAQDGDLYRLKILDLALGDSGQYVSRARNAIGEAFACVGLQVDAEA

SEQ ID NO: 212 - protein, 97 aa, synthetic construct
  DOMAIN 1..97: note = O.10
SGAPRFLTRPLAFVVSVGKDATLSSQIVGNPTPQVSWEKDQQPVAAGARFRLAQDGDLYRLHILDLALGDSGQYVSRARNAIGEAFACVGLQVDAEA

SEQ ID NO: 213 - protein, 102 aa, synthetic construct
  DOMAIN 1..102: note = O.11
DQPQFSGAPRFLTRPKAFVVSVGKDATLSSQIVGNPTPQVSWEKDQQPVAAGARFRLAQDGDLYRLTILDLALGDSGQYVSRARNAIGEAFACVGLQVDAEA

SEQ ID NO: 214 - protein, 102 aa, synthetic construct
  DOMAIN 1..102: note = O.12
DQPQFSGAPRFKTRPKAFVVSVGKDATLSSQIVGNPTPQVSWEKDQQPVAAGARFRLAQDGDLYRLKILDLALGDSGQYVSRARNAIGEAFACVGLQVDAEA

SEQ ID NO: 215 - protein, 102 aa, synthetic construct
  DOMAIN 1..102: note = O.13
DQPQFSGAPRFKTRPKAFVVSVGKDATLSSQIVGNPTPQVSWEKDQQPVAAGARFRLAQDGDLYRLHILDLALGDSGQYVSRARNAIGEAFACVGLQVDAEA

SEQ ID NO: 216 - protein, 102 aa, synthetic construct
  DOMAIN 1..102: note = O.14
DQPQFSGAPRFRTRPKAFVVSVGKDATLSSQIVGNPTPQVSWEKDQQPVAAGARFRLAQDGDLYRLKILDLALGDSGQYVSRARNAIGEAFACVGLQVDAEA

SEQ ID NO: 217 - protein, 102 aa, synthetic construct
  DOMAIN 1..102: note = O.15
DQPQFSGAPRFRTRPKAFVVSVGKDATLSSQIVGNPTPQVSWEKDQQPVAAGARFRLAQDGDLYRLHILDLALGDSGQYVSRARNAIGEAFACVGLQVDAEA

SEQ ID NO: 218 - protein, 102 aa, synthetic construct
  DOMAIN 1..102: note = O.16
DQPQFSGAPRFLTRPKAFVVSVGKDATLSCQIVGNPTPQVSWEKDQQPVAAGARFRLAQDGDLYRLTILDLALGDSGQYVCRARNAIGEAFAAVGLQVDAEA

SEQ ID NO: 219 - protein, 98 aa, synthetic construct
  DOMAIN 1..98: note = OL.1
QGSPPEFLRFPRPVRVVSGAEAELKCVVLGEPPPVVVWEKGGQQLAASERLSFPADGAEHGLLLTAALPTDAGCYVCRARNAAGEAYAAAAVTVLEPP

SEQ ID NO: 220 - protein, 98 aa, synthetic construct
  DOMAIN 1..98: note = OL.2
QGSPPEFLRFPRPVRVVSGAEAELKCVVLGEPPPVVVWEKGGQQLAASERLSFPADGAEHGLLLTAALPTDAGVYVCRARNAACEAYAAAAVTVLEPP

SEQ ID NO: 221 - protein, 98 aa, synthetic construct
  DOMAIN 1..98: note = OL.3
QGSPPEFLRFPRPVRVVSGAEAELKCVVLGEPPPVVVWEKGGQQLAASERLSFPADGAEHGLLLTAALPTDAGVYVCRARNAAGECYAAAAVTVLEPP

SEQ ID NO: 222 - protein, 98 aa, synthetic construct
  DOMAIN 1..98: note = OL.4
QGSPPEFLRFPRPVRVVSGAEAELKSVVLGEPPPVVVWEKGGQQLAASERLSFPADGAEHGLLLTAALPTDAGCYVSRARNAAGEAYAAAAVTVLEPP

SEQ ID NO: 223 - protein, 98 aa, synthetic construct
  DOMAIN 1..98: note = OL.5
QGSPPEFLRFPRPVRVVSGAEAELKSVVLGEPPPVVVWEKGGQQLAASERLSFPADGAEHGLLLTAALPTDAGVYVSRARNAACEAYAAAAVTVLEPP

SEQ ID NO: 224 - protein, 98 aa, synthetic construct
  DOMAIN 1..98: note = OL.6
QGSPPEFLRFPRPVRVVSGAEAELKSVVLGEPPPVVVWEKGGQQLAASERLSFPADGAEHGLLLTAALPTDAGVYVSRARNAAGECYAAAAVTVLEPP

SEQ ID NO: 225 - protein, 97 aa, synthetic construct
  DOMAIN 1..97: note = O.17
SGAPRFLTRPKSYTVSVGKDASLSSQIVGNPTPQVSWEKDQQPVAAGARFRLAQDGDLYRLKILDLALGDSGQYVSRARNAIGEAFACVGLQVDAEA

SEQ ID NO: 226 - protein, 97 aa, synthetic construct
  DOMAIN 1..97: note = O.18
SEAPRFLTRPLAFVVSEGKDATLSSQIVGDPPPEVTWEKDQQPITAGARFRLAQDGDVYRLEILDLQLSDSGQYVSRARNAIGEAFACVGLQVDAEG

SEQ ID NO: 227 - protein, 97 aa, synthetic construct
  DOMAIN 1..97: note = O.19
SGAPRFLTRPLAFVVSVGKLAMLSSQIVGNPTPQVSWEKDQQPVAAGARFRLLQDGDLYRLKILDLALGDSGQYVSRARNAIGEAFACVGLQVDAEA

SEQ ID NO: 228 - protein, 97 aa, synthetic construct
  DOMAIN 1..97: note = O.20
SGAPRFLTRPLAFVVSVGKDATLSSQIVGNPTPQVSWEKDKQPVTAGARFRLAQDGDLYRLKILDLQLSDSGQYVSRARNAIGEAFACLGLQVDAEA

SEQ ID NO: 229 - protein, 97 aa, synthetic construct
  DOMAIN 1..97: note = O.21
SGAPRFLTRPLAFVVSVGKDATLSSQIVGNPTPQVSWEKDQLPVTAGARFRLAQDGDLYRLKILDLTLSDSGQYVSRARNAIGEAFACVGLEVGAEA

SEQ ID NO: 230 - protein, 97 aa, synthetic construct
  DOMAIN 1..97: note = O.22
SGAPRFLTRPLSYVVSVGKDASLSSQIVGNPTPQVSWEKDQLPVTAGARFRLAQDGDLYRLKILDLQLSDSGQYVSRARNAIGEAFACVGLEVGAEA

SEQ ID NO: 231 - protein, 102 aa, synthetic construct
  DOMAIN 1..102: note = O.23
DQPQFSGAPRFLTRPLSYVVSVGKDASLSSQIVGNPTPQVSWEKDQLPVTAGARFRLAQDGDLYRLKILDLQLSDSGQYVSRARNAIGEAFACVGLEVGAEA

SEQ ID NO: 232 - protein, 97 aa, synthetic construct
  DOMAIN 1..97: note = O.24
SGAPRFLTRPKAFVVSVGKDATLSSQIVGNPFPQVSWEKDKQPVTAGVRFRLAQDGDLYRLKILDLQLSDSGQYVSRARNAIGEAFACLGLQVDAEA

SEQ ID NO: 233 - protein, 97 aa, synthetic construct
  DOMAIN 1..97: note = O.25
SGAPRFLTRPKASVVSVGKDATLSSQIVGNPFPQVSWEKDKQPVTAGVRFRLAQDGDLYRLKILDLQLSDSGQYVSRARNAHGEAFACLGLQVDAEA

SEQ ID NO: 234 - protein, 97 aa, synthetic construct
  DOMAIN 1..97: note = O.26
SGCPRFLTRPKASVVSVGKDATLSSQIVGNPFPQVSWEKDKQPVTAGVRFRLAQDGDLYRLKILDLQLSDSGQYVSRARNAHGEAFACLGLQVDAEA

SEQ ID NO: 235 - protein, 97 aa, synthetic construct
  DOMAIN 1..97: note = O.27
SGAPRFLTCPKASVVSVGKDATLSSQIVGNPFPQVSWEKDKQPVTAGVRFRLAQDGDLYRLKILDLQLSDSGQYVSRARNAHGEAFACLGLQVDAEA

SEQ ID NO: 236 - protein, 97 aa, synthetic construct
  DOMAIN 1..97: note = O.28
SGAPRFLTRPKASVVSVGKDATLSCQIVGNPFPQVSWEKDKQPVTAGVRFRLAQDGDLYRLKILDLQLSDSGQYVCRARNAHGEAFACLGLQVDAEA

SEQ ID NO: 237 - protein, 97 aa, synthetic construct
  DOMAIN 1..97: note = O.29
SGCPRFLTRPKASVVSVGKDATLSCQIVGNPFPQVSWEKDKQPVTAGVRFRLAQDGDLYRLKILDLQLSDSGQYVCRARNAHGEAFACLGLQVDAEA

SEQ ID NO: 238 - protein, 97 aa, synthetic construct
  DOMAIN 1..97: note = O.30
SGAPRFLTCPKASVVSVGKDATLSCQIVGNPFPQVSWEKDKQPVTAGVRFRLAQDGDLYRLKILDLQLSDSGQYVCRARNAHGEAFACLGLQVDAEA

SEQ ID NO: 239 - protein, 97 aa, synthetic construct
  DOMAIN 1..97: note = O.31
SGAPRFLTRPKASVVSVGKDATLSSQIVGNPFPQVSWEKDKQPVTAGVRFRLAQDGDLYRLKILDCQLSDSGQYVSRARNAHGEAFACLGLQCDAEA

SEQ ID NO: 240 - protein, 97 aa, synthetic construct
  DOMAIN 1..97: note = O.32
SGCPRFLTRPKASVVSVGKDATLSSQIVGNPFPQVSWEKDKQPVTAGVRFRLAQDGDLYRLKILDCQLSDSGQYVSRARNAHGEAFACLGLQCDAEA

SEQ ID NO: 241 - protein, 97 aa, synthetic construct
  DOMAIN 1..97: note = O.33
SGAPRFLTCPKASVVSVGKDATLSSQIVGNPFPQVSWEKDKQPVTAGVRFRLAQDGDLYRLKILDCQLSDSGQYVSRARNAHGEAFACLGLQCDAEA

SEQ ID NO: 242 - protein, 455 aa, synthetic construct
  CHAIN 1..455: note = Format 2-1 (N103QN106Q)
EVQLVESGGGLVQPGGSLKLSCAASGFTFNKYAMNWVRQAPGKGLEWVARIRSKYNNYATYYADSVKDRFTISRDDSKNTAYLQMNNLKTEDTAVYYCVRHGQFGQSYISYWAYWGQGTLVTVSSASTKGPSVFPLAPSSKSTSGGTAALGCLVKDYFPEPVTVSWNSGALTSGVHTFPAVLQSSGLYSLSSVVTVPSSSLGTQTYICNVNHKPSNTKVDKKVEPKSCDKTHTCPPCPAPEAAGGPSVFLFPPKPKDTLMISRTPEVTCVVVDVSHEDPEVKFNWYVDGVEVHNAKTKPREEQYNSTYRVVSVLTVLHQDWLNGKEYKCKVSNKALPAPIEKTISKAKGQPREPQVYTLPPCREEMTKNQVSLWCLVKGFYPSDIAVEWESNGQPENNYKTTPPVLDSDGSFFLYSKLTVDKSRWQQGNVFSCSVMHEALHNHYTQKSLSLSPGK

SEQ ID NO: 243 - protein, 5 aa, synthetic construct
  DOMAIN 1..5: note = linker
ASTKG

SEQ ID NO: 244 - protein, 5 aa, synthetic construct
RTVAS

SEQ ID NO: 245 - skipped

SEQ ID NO: 246 - protein, 4 aa, synthetic construct
  DOMAIN 1..4: note = linker
GGGS

SEQ ID NO: 247 - protein, 4 aa, synthetic construct
  DOMAIN 1..4: note = linker
GGGG

SEQ ID NO: 248 - protein, 227 aa, synthetic construct
  DOMAIN 1..227: note = IgG1Fc-Knob L234A/L235A/S354C/T366W
DKTHTCPPCPAPEAAGGPSVFLFPPKPKDTLMISRTPEVTCVVVDVSHEDPEVKFNWYVDGVEVHNAKTKPREEQYNSTYRVVSVLTVLHQDWLNGKEYKCKVSNKALPAPIEKTISKAKGQPREPQVYTLPPCRDELTKNQVSLWCLVKGFYPSDIAVEWESNGQPENNYKTTPPVLDSDGSFFLYSKLTVDKSRWQQGNVFSCSVMHEALHNHYTQKSLSLSPGK

SEQ ID NO: 249 - protein, 227 aa, synthetic construct
  DOMAIN 1..227: note = IgG1Fc-Hole L234A/L235A/Y349C/T366S/L368A/Y407V
DKTHTCPPCPAPEAAGGPSVFLFPPKPKDTLMISRTPEVTCVVVDVSHEDPEVKFNWYVDGVEVHNAKTKPREEQYNSTYRVVSVLTVLHQDWLNGKEYKCKVSNKALPAPIEKTISKAKGQPREPQVCTLPPSRDELTKNQVSLSCAVKGFYPSDIAVEWESNGQPENNYKTTPPVLDSDGSFFLVSKLTVDKSRWQQGNVFSCSVMHEALHNHYTQKSLSLSPGK

SEQ ID NO: 250 - protein, 5 aa, synthetic construct
  DOMAIN 1..5: note = M42-HCDR1
SYAVH

SEQ ID NO: 251 - protein, 16 aa, synthetic construct
  DOMAIN 1..16: note = M42-HCDR2
VIWTGGNTRSNAAFMS

SEQ ID NO: 252 - protein, 10 aa, synthetic construct
  DOMAIN 1..10: note = M42-HCDR3
NSLLDYAMDY

SEQ ID NO: 253 - protein, 12 aa, synthetic construct
  DOMAIN 1..12: note = M42-LCDR1
RASSFVGSGYLH

SEQ ID NO: 254 - protein, 7 aa, synthetic construct
  DOMAIN 1..7: note = M42-LCDR2
STSKLAS

SEQ ID NO: 255 - protein, 9 aa, synthetic construct
  DOMAIN 1..9: note = M42-LCDR3
QQSSGYPLT

SEQ ID NO: 256 - protein, 5 aa, synthetic construct
  DOMAIN 1..5: note = M61-HCDR1
DYYMS

SEQ ID NO: 257 - protein, 17 aa, synthetic construct
  DOMAIN 1..17: note = M61-HCDR2
DINPNNGGTSDNQKFKG

SEQ ID NO: 258 - protein, 11 aa, synthetic construct
  DOMAIN 1..11: note = M61-HCDR3
GRGMVARYFDI

SEQ ID NO: 259 - protein, 12 aa, synthetic construct
  DOMAIN 1..12: note = M61-LCDR1
SASSSISSNFLH

SEQ ID NO: 260 - protein, 9 aa, synthetic construct
  DOMAIN 1..9: note = M61-LCDR3
QQGSGLPLT

SEQ ID NO: 261 - protein, 5 aa, synthetic construct
  DOMAIN 1..5: note = M64-HCDR1
DYGMH

SEQ ID NO: 262 - protein, 17 aa, synthetic construct
  DOMAIN 1..17: note = M64-HCDR2
YISSGSSTIYYADTVKG

SEQ ID NO: 263 - protein, 14 aa, synthetic construct
  DOMAIN 1..14: note = M64-HCDR3
TRVYFYGSYWYFDV

SEQ ID NO: 264 - protein, 10 aa, synthetic construct
  DOMAIN 1..10: note = M64-LCDR1
SASSSVSYMY

SEQ ID NO: 265 - protein, 7 aa, synthetic construct
  DOMAIN 1..7: note = M64-LCDR2
DTSKLAS

SEQ ID NO: 266 - protein, 10 aa, synthetic construct
  DOMAIN 1..10: note = M64-LCDR3
QQWSSDPPYT

SEQ ID NO: 267 - protein, 5 aa, synthetic construct
  DOMAIN 1..5: note = M93-HCDR1
RYWMH

SEQ ID NO: 268 - protein, 17 aa, synthetic construct
  DOMAIN 1..17: note = M93-HCDR2
MIDPSDSYTKYNQKFMG

SEQ ID NO: 269 - protein, 11 aa, synthetic construct
  DOMAIN 1..11: note = M93-HCDR3
SIKVAGWYFDV

SEQ ID NO: 270 - protein, 11 aa, synthetic construct
  DOMAIN 1..11: note = M93-LCDR1
KASQDVSSAVA

SEQ ID NO: 271 - protein, 7 aa, synthetic construct
  DOMAIN 1..7: note = M93-LCDR2
SASYRST

SEQ ID NO: 272 - protein, 9 aa, synthetic construct
  DOMAIN 1..9: note = M93-LCDR3
QQHFSTTLT

SEQ ID NO: 273 - protein, 118 aa, synthetic construct
  DOMAIN 1..118: note = M42VH
QIQLKQSGPGLVQPSQSLSITCTVSGFSLTSYAVHWVRQSPGKGLEWLGVIWTGGNTRSNAAFMSRLTITKDNSKSQVFFKMNSLQADDTAIYFCAKNSLLDYAMDYWGQGTSVTVSS

SEQ ID NO: 274 - protein, 108 aa, synthetic construct
  DOMAIN 1..108: note = M42VL
ENVLTQSPVIMSASPGEKVTMTCRASSFVGSGYLHWYQQKSGASPKLWIYSTSKLASGVPARFSGSGSGTSFFLTISRVEIEDAAAYYCQQSSGYPLTFGGGSKLEIK

SEQ ID NO: 275 - protein, 120 aa, synthetic construct
  DOMAIN 1..120: note = M61VH
EVQLQQSGPELVRPGASVKISCTASGYTITDYYMSWVKQSHGKSPEWIGDINPNNGGTSDNQKFKGKATLTVDKSSSTAYMEYRSLTSEDSAVYYCARGRGMVARYFDIWGTGTTVTVSS

SEQ ID NO: 276 - protein, 108 aa, synthetic construct
  DOMAIN 1..108: note = M61VL
EILLTQSPTTMAASPGEKITITCSASSSISSNFLHWYQEKPGFSPKLLIYRTSNLASGVPARFSGSGSGTSYSLTIGSMEAEDVATYYCQQGSGLPLTFGAGTKLELK

SEQ ID NO: 277 - protein, 123 aa, synthetic construct
  DOMAIN 1..123: note = M64VH
EVQLVESGGGLVKPGGSLKLSCAASGFTFSDYGMHWVRQAPEKGLEWVAYISSGSSTIYYADTVKGRFTISRDNAKNTLFLQMTSLRSEDTAMYYCARTRVYFYGSYWYFDVWGTGTTVTVSS

SEQ ID NO: 278 - protein, 107 aa, synthetic construct
  DOMAIN 1..107: note = M64VL
QIVLTQSPAIMSASPGEKVTMTCSASSSVSYMYWYQQKSGTSPKRWIYDTSKLASGVPARFSGSGSGTSYSLTISSLEAEDAATYYCQQWSSDPPYTFGGGTKLEIK

SEQ ID NO: 279 - protein, 120 aa, synthetic construct
  DOMAIN 1..120: note = M93VH
QVQLQQPGAELVRPGTSVKLSCKASGYTFTRYWMHGVKRRPGQGLEWIGMIDPSDSYTKYNQKFMGKAILTVDTSSSTAYMQFSSLTSEDSAVYYCARSIKVAGWYFDVWGTGTTVTVSS

SEQ ID NO: 280 - protein, 107 aa, synthetic construct
  DOMAIN 1..107: note = M93VL
DIVMTQSHKFMSTSVGDRVSITCKASQDVSSAVAWYQQKPGQSPKLLIYSASYRSTGVPDRFTGSGSGTDFTFTISSVQAEDLAIYYCQQHFSTTLTFGAGTKLELK

SEQ ID NO: 281 - protein, 5 aa, synthetic construct
  DOMAIN 1..5: note = P1-D2-HCDR1
DHNMN

SEQ ID NO: 282 - protein, 17 aa, synthetic construct
  DOMAIN 1..17: note = P1-D2-HCDR2
VINPKYGTISNNQKFKG

SEQ ID NO: 283 - protein, 9 aa, synthetic construct
  DOMAIN 1..9: note = P1-D2-HCDR3
DDYPNYFDY

SEQ ID NO: 284 - protein, 10 aa, synthetic construct
  DOMAIN 1..10: note = P1-D2-LCDR1
SANSSVNYIY

SEQ ID NO: 285 - protein, 9 aa, synthetic construct
  DOMAIN 1..9: note = P1-D2-LCDR3
QQYHSFPPT

SEQ ID NO: 286 - protein, 5 aa, synthetic construct
  DOMAIN 1..5: note = P1-D3-HCDR1
TYGMS

SEQ ID NO: 287 - protein, 17 aa, synthetic construct
  DOMAIN 1..17: note = P1-D3-HCDR2
WINTYSGVPTYADDFKG

SEQ ID NO: 288 - protein, 13 aa, synthetic construct
  DOMAIN 1..13: note = P1-D3-HCDR3
RGYSNLYYYALDY

SEQ ID NO: 289 - protein, 10 aa, synthetic construct
  DOMAIN 1..10: note = P1-D3-LCDR1
SASSSVNYMH

SEQ ID NO: 290 - protein, 9 aa, synthetic construct
  DOMAIN 1..9: note = P1-D3-LCDR3
QQWSSNPST

SEQ ID NO: 291 - protein, 5 aa, synthetic construct
  DOMAIN 1..5: note = P1-C6-HCDR1
SYGIT

SEQ ID NO: 292 - protein, 17 aa, synthetic construct
  DOMAIN 1..17: note = P1-C6-HCDR2
EIYPRSGNTYYNEKFKG

SEQ ID NO: 293 - protein, 13 aa, synthetic construct
  DOMAIN 1..13: note = P1-C6-HCDR3
AITTVVGDWYFDV

SEQ ID NO: 294 - protein, 15 aa, synthetic construct
  DOMAIN 1..15: note = P1-C6-LCDR1
RASESVSLIGTNLIH

SEQ ID NO: 295 - protein, 7 aa, synthetic construct
  DOMAIN 1..7: note = P1-C6-LCDR2
HASNLEA

SEQ ID NO: 296 - protein, 8 aa, synthetic construct
  DOMAIN 1..8: note = P1-C6-LCDR3
LQSRKIRT

SEQ ID NO: 297 - protein, 17 aa, synthetic construct
  DOMAIN 1..17: note = P1-D9-HCDR2
HISSGSSTIYYADTVKG

SEQ ID NO: 298 - protein, 12 aa, synthetic construct
  DOMAIN 1..12: note = P1-D9-HCDR3
SRNYYGSRIFDY

SEQ ID NO: 299 - protein, 7 aa, synthetic construct
  DOMAIN 1..7: note = P1-D9-LCDR2
LTSNLAS

SEQ ID NO: 300 - protein, 9 aa, synthetic construct
  DOMAIN 1..9: note = P1-D9-LCDR3
QQWSSNPPT

SEQ ID NO: 301 - protein, 17 aa, synthetic construct
  DOMAIN 1..17: note = P1-F10-HCDR2
HISSGSSTIYYADTVKG

SEQ ID NO: 302 - protein, 12 aa, synthetic construct
  DOMAIN 1..12: note = P1-F10-HCDR3
SRNYYGSRVFDY

SEQ ID NO: 303 - protein, 10 aa, synthetic construct
  DOMAIN 1..10: note = P1-F10-LCDR1
SASSSVNYMY

SEQ ID NO: 304 - protein, 9 aa, synthetic construct
  DOMAIN 1..9: note = P1-F10-LCDR3
QQWNSNPPT

SEQ ID NO: 305 - protein, 5 aa, synthetic construct
  DOMAIN 1..5: note = P2-C8-HCDR1
DYYMH

SEQ ID NO: 306 - protein, 17 aa, synthetic construct
  DOMAIN 1..17: note = P2-C8-HCDR2
LINPYNGVTSYNQKFKG

SEQ ID NO: 307 - protein, 17 aa, synthetic construct
  DOMAIN 1..17: note = P2-B9-HCDR2
MIHPKSDSVNNNEKFKN

SEQ ID NO: 308 - protein, 10 aa, synthetic construct
  DOMAIN 1..10: note = P2-B9-HCDR3
GGDSGYSMDY

SEQ ID NO: 309 - protein, 16 aa, synthetic construct
  DOMAIN 1..16: note = P2-B9-LCDR1
KASKKVTIFGSISALH

SEQ ID NO: 310 - protein, 7 aa, synthetic construct
  DOMAIN 1..7: note = P2-B9-LCDR2
NGAKLES

SEQ ID NO: 311 - protein, 9 aa, synthetic construct
  DOMAIN 1..9: note = P2-B9-LCDR3
LQNKEVPYT

SEQ ID NO: 312 - protein, 5 aa, synthetic construct
  DOMAIN 1..5: note = P3-D2-HCDR1
DYFMH

SEQ ID NO: 313 - protein, 17 aa, synthetic construct
  DOMAIN 1..17: note = P3-D2-HCDR2
LINPYSGGTTYNQKFKG

SEQ ID NO: 314 - protein, 11 aa, synthetic construct
  DOMAIN 1..11: note = P3-D2-HCDR3
PPRAYGDYAGY

SEQ ID NO: 315 - protein, 9 aa, synthetic construct
  DOMAIN 1..9: note = P3-D2-LCDR3
SQSTHVPLT

SEQ ID NO: 316 - protein, 13 aa, synthetic construct
  DOMAIN 1..13: note = P3-B4-HCDR3
RAGSSLYYYAMDY

SEQ ID NO: 317 - protein, 10 aa, synthetic construct
  DOMAIN 1..10: note = P3-B4-LCDR1
SASSSVSYML

SEQ ID NO: 318 - protein, 5 aa, synthetic construct
  DOMAIN 1..5: note = P3-E4-HCDR1
NYWMH

SEQ ID NO: 319 - protein, 17 aa, synthetic construct
  DOMAIN 1..17: note = P3-E4-HCDR2
EIDPSDGYTDYNQKFKG

SEQ ID NO: 320 - protein, 13 aa, synthetic construct
  DNA_BIND 1..13: note = P3-E4-HCDR3
SLRGPITFGPFPY

SEQ ID NO: 321 - protein, 15 aa, synthetic construct
  DOMAIN 1..15: note = P3-E4-LCDR1
RASESVSIHGTHLMH

SEQ ID NO: 322 - protein, 7 aa, synthetic construct
  DOMAIN 1..7: note = P3-E4-LCDR2
AASNLES

SEQ ID NO: 323 - protein, 9 aa, synthetic construct
  DOMAIN 1..9: note = P3-E4-LCDR3
QHSIEDPRT

SEQ ID NO: 324 - protein, 5 aa, synthetic construct
  DOMAIN 1..5: note = P3-F6-HCDR1
DYYMN

SEQ ID NO: 325 - protein, 17 aa, synthetic construct
  DOMAIN 1..17: note = P3-F6-HCDR2
DINPNNGGTSYNQKFKG

SEQ ID NO: 326 - protein, 10 aa, synthetic construct
  DOMAIN 1..10: note = P3-F6-HCDR3
KTWLPYASVY

SEQ ID NO: 327 - protein, 10 aa, synthetic construct
  DOMAIN 1..10: note = P3-F6-LCDR3
SQSTHVPPYT

SEQ ID NO: 328 - protein, 17 aa, synthetic construct
  DOMAIN 1..17: note = P3-D9-HCDR2
HISSGSSTIYYGDTVKG

SEQ ID NO: 329 - protein, 7 aa, synthetic construct
  DOMAIN 1..7: note = P3-D9-LCDR2
LTSSLAS

SEQ ID NO: 330 - protein, 118 aa, synthetic construct
  DOMAIN 1..118: note = P1-D2 VH
EFQLQQSGPELVKPGASVKISCKASGYSFTDHNMNWVKQSNGKSLEWIGVINPKYGTISNNQKFKGKATLTVDQSSSTAYMQLNSLTAEDSAVYYCARDDYPNYFDYWGQGTTLTVSS

SEQ ID NO: 331 - protein, 106 aa, synthetic construct
  DOMAIN 1..106: note = P1-D2 VL
QIVLTQSPAIMSASPGEKVTISCSANSSVNYIYWYQQKPGSSPKPWIYRTSNLASGVPARFSGSGSGTSYSLTISSMEAEDAATYYCQQYHSFPPTFGGGTKLEIK

SEQ ID NO: 332 - protein, 122 aa, synthetic construct
  DOMAIN 1..122: note = P1-D3 VH
QIQLIQSGPELKKPGETVKISCKASGYTFTTYGMSWVKQAPGKGLKWMGWINTYSGVPTYADDFKGRFAFSLETSANTAYLQINNLKNEDTATYFCARRGYSNLYYYALDYWGQGASVTVSS

SEQ ID NO: 333 - protein, 106 aa, synthetic construct
  DOMAIN 1..106: note = P1-D3 VL
QIVLTQSPAIMSASPGEKVTMTCSASSSVNYMHWYQQKSGTSPKRWIYDTSKLASGVPTRFSGSGSGTSYSLTISSMEAEDAATYFCQQWSSNPSTFGGGTKLEIK

SEQ ID NO: 334 - protein, 122 aa, synthetic construct
  DOMAIN 1..122: note = P1-C6 VH
QVQLQQSGAELARPGASVKLSCKASGYTFTSYGITWVKRRTGQGLGWIGEIYPRSGNTYYNEKFKGKATLTADKSSSTAYMELRSLTSEDSAVYFCARAITTVVGDWYFDVWGTGTTVTVSS

SEQ ID NO: 335 - protein, 110 aa, synthetic construct
  DOMAIN 1..110: note = P1-C6 VL
DIVLTQSPASLAMSLGKRATISCRASESVSLIGTNLIHWYQQKPGQPPKLLIHHASNLEAGVPARFSGSGSRTDFTLTIDPVEEDDVAIYYCLQSRKIRTFGGGTKLEIK

SEQ ID NO: 336 - protein, 121 aa, synthetic construct
  DOMAIN 1..121: note = P1-D9 VH
EVQLVESGGGLVKPGGSLKLSCAASGFSFSDYGMHWVRQAPEKGLEWIAHISSGSSTIYYADTVKGRFTISRDNAKNTLFLQMTSLRSEDTAMYYCARSRNYYGSRIFDYWGQGTTLTVSS

SEQ ID NO: 337 - protein, 106 aa, synthetic construct
  DOMAIN 1..106: note = P1-D9 VL
QIVLTQSPARMSASPGEKVTMTCSASSSVSYMYWYQQKPRSSPKPWIYLTSNLASGVPARFSGSGSGTSYSLTISSMEAEDAATYYCQQWSSNPPTFGSGTKLEIK

SEQ ID NO: 338 - protein, 121 aa, synthetic construct
  DOMAIN 1..121: note = P1-F10 VH
EVQLVESGGGLVKPGGSLKLSCAASGFAFSDYGMHWVRQAPEKGLEWVAHISSGSSTIYYADTVKGRFTISRDNVKNTLFLQMTSLRSEDTAMYYCARSRNYYGSRVFDYWGQGTPLTVSS

SEQ ID NO: 339 - protein, 106 aa, synthetic construct
  DOMAIN 1..106: note = P1-F10 VL
QIVLTQSPALMSVSPGEKVTMTCSASSSVNYMYWYQQKPRSSPKPWIYLTSNLASGVPARFSGSGSGTSYSLTISSMEAEDAATYYCQQWNSNPPTFGSGTKLEIK

SEQ ID NO: 340 - protein, 120 aa, synthetic construct
  DOMAIN 1..120: note = P2-C8 VH
EVQLQQSGPVLVKPGASVKMSCKVSGYTFTDYYMHWVKQSHGKSLEWIGLINPYNGVTSYNQKFKGKATLTVDKSSSTAYMELNSLTSEDSAVYYCARPPRAYGNYAGYWGQGTTLTVSS

SEQ ID NO: 341 - protein, 112 aa, synthetic construct
  DOMAIN 1..112: note = P2-C8 VL
DVVMTQTPLSLPVSLGDQASISCRSSQSLVHSNGNTYLHWYLQKPGQSPKLLIYKVSNRFSGVPDRFSGSGSGTDFTLKISRVEAEDLGVYFCSQSTHVPYTFGGGTKLEIK

SEQ ID NO: 342 - protein, 119 aa, synthetic construct
  DOMAIN 1..119: note = P2-B9 VH
QVQLQQPGAELVKPGASVKLSCKASGYTFSSYWMHWVKQRPGQGLEWIGMIHPKSDSVNNNEKFKNKATLTVDKSSSTVYLQLSSLTSEDSAVYSCARGGDSGYSMDYWGQGTSVTVSS

SEQ ID NO: 343 - protein, 119 aa, synthetic construct
  DOMAIN 1..119: note = P2-B9 VL
DIVLTQSPASLAVSLGQKATISCKASKKVTIFGSISALHWYQQKPGQPPKLIYNGAKLESGVSARFSDSGSQNRSPFGNQLSFTLTIDPVEADDAATYYCLQNKEVPYTFGGGTKLEIK

SEQ ID NO: 344 - protein, 120 aa, synthetic construct
  DOMAIN 1..120: note = P3-D2 VH
EVQLQQSGPVLVKPGASVKMSCKASGYTFTDYFMHWVKQSHGKSLEWIGLINPYSGGTTYNQKFKGKATLTVDKSSSTAYMELNSLTSEDSAVYYCARPPRAYGDYAGYWGQGTTLTVSS

SEQ ID NO: 345 - protein, 112 aa, synthetic construct
  DOMAIN 1..112: note = P3-D2 VL
DVVMTQTPLSLPVSLGDQASISCRSSQSLVHSNGNTYLHWYLQKPGQSPKLLIYKVSNRFSGVPDRFSGSGSGTDFTLKISRVEAEDLGVYFCSQSTHVPLTFGTGTKLEIK

SEQ ID NO: 346 - protein, 122 aa, synthetic construct
  DOMAIN 1..122: note = P3-B4 VH
QIQLVQSGPELKKPGEIVKISCKASGYTFTTYGMSWVKQAPGKGLKWMGWINTYSGVPTYADDFKGRFAFSLETSASTAYLQINNLKNEDTATYFCARRAGSSLYYYAMDYWGQGTSVTVSS

SEQ ID NO: 347 - protein, 106 aa, synthetic construct
  DOMAIN 1..106: note = P3-B4 VL
QIVLTQSPAIMSASPGEKVTMTCSASSSVSYMLWYQQKSGTSPKRWIYDTSKLASGVPARFSGSGSGTSYSLTISSMEAEDAATYYCQQWSSNPPTFGGGTKLEIK

SEQ ID NO: 348 - protein, 122 aa, synthetic construct
  DOMAIN 1..122: note = P3-E4 VH
QVQLQQPGAELVMPGAAVKLSCKASGYTFINYWMHWLKQRPGQGLEWIGEIDPSDGYTDYNQKFKGKATLTVDKSSSTAYMQLSSLTSEDSAVYYCAISLRGPITFGPFPYWGQGTLVTVSS

SEQ ID NO: 349 - protein, 111 aa, synthetic construct
  DOMAIN 1..111: note = P3-E4 VL
DIVLTQSPASLAVSLGQRATISCRASESVSIHGTHLMHWYQQKPGQPPKLLIYAASNLESGVPARFSGSGSETDFTLNIHPVAEEDAATYFCQHSIEDPRTFGGGTKLEIK

SEQ ID NO: 350 - protein, 119 aa, synthetic construct
  DOMAIN 1..119: note = P3-F6 VH
EVQLQQSGPELVKPGASVKISCKASGYTFTDYYMNWVKQSHGKSLEWIGDINPNNGGTSYNQKFKGKATLTVDKSSSTAYMELRSLTSEDSAVYYCARKTWLPYASVYWGQGTSVTVSS

SEQ ID NO: 351 - protein, 113 aa, synthetic construct
  DOMAIN 1..113: note = P3-F6 VL
DVVMTQTPLSLPVSLGDQASISCRSSQSLVHSNGNTYLHWYLQKPGQSPKLLIYKVSNRFSGVPDRFSGSGSGTDFTLKISRVEAEDLGVYFCSQSTHVPPYTFGGGTKLEIK

SEQ ID NO: 352 - protein, 121 aa, synthetic construct
  DOMAIN 1..121: note = P3-D9 VH
EVQLVESGGGLVKPGGSLKLSCAASGFAFSDYGMHWVRQAPEKGLEWVAHISSGSSTIYYGDTVKGRFTISRDNAKNTLFLQMTSLRSEDTAMYYCTRSRNYYGSRVFDYWGQGTTLTVSS

SEQ ID NO: 353 - protein, 106 aa, synthetic construct
  DOMAIN 1..106: note = P3-D9 VL
QIVLTQSPALMSVSPGEKVTMTCSASSSVSYMYWYQQKPRSSPKPWIYLTSSLASGVPARFSGSGSGTSYSLTINNVEAEDAATYYCQQWSSNPPTFGSGTKVEIK

SEQ ID NO: 354 - protein, 448 aa, synthetic construct
  CHAIN 1..448: note = M81CHI-heavy chain
EFQLQQSGPELVKPGASVKISCKASGYSFTDHNMNWVKQSNGKSLEWIGVMNPKFGTINYNQKFKDKATLTVDQSSSTAYMQLNSLTSEDSAVYYCVRDDYPNYFDYWGQGTTLTVSSASTKGPSVFPLAPSSKSTSGGTAALGCLVKDYFPEPVTVSWNSGALTSGVHTFPAVLQSSGLYSLSSVVTVPSSSLGTQTYICNVNHKPSNTKVDKKVEPKSCDKTHTCPPCPAPELLGGPSVFLFPPKPKDTLMISRTPEVTCVVVDVSHEDPEVKFNWYVDGVEVHNAKTKPREEQYNSTYRVVSVLTVLHQDWLNGKEYKCKVSNKALPAPIEKTISKAKGQPREPQVYTLPPSRDELTKNQVSLTCLVKGFYPSDIAVEWESNGQPENNYKTTPPVLDSDGSFFLYSKLTVDKSRWQQGNVFSCSVMHEALHNHYTQKSLSLSPGK

SEQ ID NO: 355 - protein, 213 aa, synthetic construct
  DOMAIN 1..213: note = M81CHI-light chain
QIVLTQSPAIMSASPGEKVTISCSASSSVNYMYWYQQKPGSSPKSWIYRTSNLASGVSARFSGSGSGTSYSLTISSMEAEDAATYYCQQYHDYPPTFGGGTKLEIKRTVAAPSVFIFPPSDEQLKSGTASVVCLLNNFYPREAKVQWKVDNALQSGNSQESVTEQDSKDSTYSLSSTLTLSKADYEKHKVYACEVTHQGLSSPVTKSFNRGEC

SEQ ID NO: 356 - protein, 450 aa, synthetic construct
  CHAIN 1..450: note = P3-C7 CHI-heavy chain
EVQLQQSGPVLLKPGASVKMSCKASGYTFTDHYIHWVKLSHGKSLEWIGVINPYNDGATYNQKFKGKATLTVDKSSSTAYMELNSLTSEDSAVYYCARPPRAYGNYAGYWGQGTTLTVSSASTKGPSVFPLAPSSKSTSGGTAALGCLVKDYFPEPVTVSWNSGALTSGVHTFPAVLQSSGLYSLSSVVTVPSSSLGTQTYICNVNHKPSNTKVDKKVEPKSCDKTHTCPPCPAPELLGGPSVFLFPPKPKDTLMISRTPEVTCVVVDVSHEDPEVKFNWYVDGVEVHNAKTKPREEQYNSTYRVVSVLTVLHQDWLNGKEYKCKVSNKALPAPIEKTISKAKGQPREPQVYTLPPSRDELTKNQVSLTCLVKGFYPSDIAVEWESNGQPENNYKTTPPVLDSDGSFFLYSKLTVDKSRWQQGNVFSCSVMHEALHNHYTQKSLSLSPGK

SEQ ID NO: 357 - protein, 219 aa, synthetic construct
  DOMAIN 1..219: note = P3-C7 CHI-light chain
DVVMTQTPLSLPVSLGDQASISCRSSQSLVHSNGNTYLHWYLQKPGQSPKLLIYKVSNRFSGVPDRFIGSGSRTDFTLKISRVEAEDLGVYFCSQSTHVPYTFGGGTRLEIKRTVAAPSVFIFPPSDEQLKSGTASVVCLLNNFYPREAKVQWKVDNALQSGNSQESVTEQDSKDSTYSLSSTLTLSKADYEKHKVYACEVTHQGLSSPVTKSFNRGEC